European Patent Application EP 4 374 916 A2, published May 29, 2024. Title: A NOVEL IL33 FORM, MUTATED FORMS OF IL33, ANTIBODIES, ASSAYS AND METHODS OF USING THE SAME. Applicant: MedImmune Limited. Application EP. The sequence listing filed with the application follows.

SEQUENCE LISTING (650 sequences)

SEQ ID NO: 1 - DNA, 372 bp, synthetic construct
  misc_feature 1..372: note = Homo sapiensIL330002 VH DNA
  source 1..372: mol_type = other DNA
gaggtgcagctgttggagtctgggggaggcttggtacagcctggggggtccctgagactctcctgtgcagcctctggattcacctttagcagctatgccatgagctgggtccgccaggctccagggaaggggctggagtgggtctcagctattagtggtagtggtggtagcacatactacgcagactccgtgaagggccggttcaccatctccagagacaattccaagaacacgctgtatctgcaaatgaacagcctgagagccgaggacacggccgtgtattactgtgcgagagagtcgtattacgatttttggagtggccaatattactttgattactgggggcgggggaccacggtcaccgtctcgagt

SEQ ID NO: 2 - protein, 124 aa, synthetic construct
  REGION 1..124: note = Homo sapiensIL330002 VH PRT
EVQLLESGGGLVQPGGSLRLSCAASGFTFSSYAMSWVRQAPGKGLEWVSAISGSGGSTYYADSVKGRFTISRDNSKNTLYLQMNSLRAEDTAVYYCARESYYDFWSGQYYFDYWGRGTTVTVSS

SEQ ID NO: 3 - protein, 5 aa, synthetic construct
  REGION 1..5: note = Homo sapiensIL330002 VH CDR1 PRT
SYAMS

SEQ ID NO: 4 - protein, 17 aa, synthetic construct
  REGION 1..17: note = Homo sapiensIL330002 VH CDR2 PRT
AISGSGGSTYYADSVKG

SEQ ID NO: 5 - protein, 15 aa, synthetic construct
  REGION 1..15: note = Homo sapiensIL330002 VH CDR3 PRT
ESYYDFWSGQYYFDY

SEQ ID NO: 6 - DNA, 321 bp, synthetic construct
  misc_feature 1..321: note = Homo sapiensIL330002 VL DNA
  source 1..321: mol_type = other DNA
tcctatgagctgactcagccaccctcattgtccgtgtccccaggacagacagccagcatcacctgctctggagataaattgggagataaatatgtttcctggtatcaacagaagccaggccagtcccctatcctggtcatctatcacgataacaagcggccctcagggatccctgagcgattctctggctccaactctgggaacacagccactctgaccatcagcgggacccaggctatggatgaggctgactattactgtcaggcgtgggacagtaacgctggatatgtcttcggaactgggaccaaggtcaccgtccta

SEQ ID NO: 7 - protein, 107 aa, synthetic construct
  REGION 1..107: note = Homo sapiensIL330002 VL PRT
SYELTQPPSLSVSPGQTASITCSGDKLGDKYVSWYQQKPGQSPILVIYHDNKRPSGIPERFSGSNSGNTATLTISGTQAMDEADYYCQAWDSNAGYVFGTGTKVTVL

SEQ ID NO: 8 - protein, 11 aa, synthetic construct
  REGION 1..11: note = Homo sapiensIL330002 VL CDR1 PRT
SGDKLGDKYVS

SEQ ID NO: 9 - protein, 7 aa, synthetic construct
  REGION 1..7: note = Homo sapiensIL330002 VL CDR2 PRT
HDNKRPS

SEQ ID NO: 10 - protein, 10 aa, synthetic construct
  REGION 1..10: note = Homo sapiensIL330002 VL CDR3 PRT
QAWDSNAGYV

SEQ ID NO: 11 - DNA, 372 bp, synthetic construct
  misc_feature 1..372: note = Homo sapiensIL330004 VH DNA
  source 1..372: mol_type = other DNA
gaggtgcagctgttggagtctgggggaggcttggtacagcctggggggtccctgagactctcctgtgcagcctctggattcacctttagcagctatgccatgagctgggtccgccaggctccagggaaggggctggagtgggtctcagctattagtggtagtggtggtagcacatactacgcagactccgtgaagggccggttcaccatctccagagacaattccaagaacacgctgtatctgcaaatgaacagcctgagagccgaggacacggccgtgtattactgtgcgagagagtcgtattacgatttttggagtggccaatattactttgattactggggccaagggacaatggtcaccgtctcgagt

SEQ ID NO: 12 - protein, 124 aa, synthetic construct
  REGION 1..124: note = Homo sapiensIL330004 VH PRT
EVQLLESGGGLVQPGGSLRLSCAASGFTFSSYAMSWVRQAPGKGLEWVSAISGSGGSTYYADSVKGRFTISRDNSKNTLYLQMNSLRAEDTAVYYCARESYYDFWSGQYYFDYWGQGTMVTVSS

SEQ ID NO: 13 - protein, 5 aa, synthetic construct
  REGION 1..5: note = Homo sapiensIL330004 VH CDR1 PRT
SYAMS

SEQ ID NO: 14 - protein, 17 aa, synthetic construct
  REGION 1..17: note = Homo sapiensIL330004 VH CDR2 PRT
AISGSGGSTYYADSVKG

SEQ ID NO: 15 - protein, 15 aa, synthetic construct
  REGION 1..15: note = Homo sapiensIL330004 VH CDR3 PRT
ESYYDFWSGQYYFDY

SEQ ID NO: 16 - DNA, 318 bp, synthetic construct
  misc_feature 1..318: note = Homo sapiensIL330004 VL DNA
  source 1..318: mol_type = other DNA
tcctatgagctgactcagccaccctcagtgtccgtgtccccaggacagactgccagcatctcctgctctggagataaattgggggataaatttgcttcctggtatcagcaaaagccaggccagtcccctgtcttgatcatctatcaggataggaagcggccctcaggaatccctgagcggttctctggctccaactctgggaacacagccactctgaccatcagcgggacccagactaccgatgaggctgactattactgtcaggcgtgggacggcagcctttatgtcttcggaactgggaccaagctgaccgtccta

SEQ ID NO: 17 - protein, 106 aa, synthetic construct
  REGION 1..106: note = Homo sapiensIL330004 VL PRT
SYELTQPPSVSVSPGQTASISCSGDKLGDKFASWYQQKPGQSPVLIIYQDRKRPSGIPERFSGSNSGNTATLTISGTQTTDEADYYCQAWDGSLYVFGTGTKLTVL

SEQ ID NO: 18 - protein, 11 aa, synthetic construct
  REGION 1..11: note = Homo sapiensIL330004 VL CDR1 PRT
SGDKLGDKFAS

SEQ ID NO: 19 - protein, 7 aa, synthetic construct
  REGION 1..7: note = Homo sapiensIL330004 VL CDR2 PRT
QDRKRPS

SEQ ID NO: 20 - protein, 9 aa, synthetic construct
  REGION 1..9: note = Homo sapiensIL330004 VL CDR3 PRT
QAWDGSLYV

SEQ ID NO: 21 - DNA, 369 bp, synthetic construct
  misc_feature 1..369: note = Homo sapiensIL330020 VH DNA
  source 1..369: mol_type = other DNA
caggtgcagctggtgcagtctggagctgaggtgaagaagcctggggcctcagtgaaggtctcctgcaaggcttctggttacacctttaccagctacggtatcagctgggtgcgacaggcccctggacaagggcttgagtggatgggatggatcagcgattaccagggttatacaaagtatgcagagaagttccagggcagagtcaccatgaccacagacacatccacgaacacagcctacatggagctgaggagcctgagatctgacgacacggccgtgtattactgtgcgagactgtatagcagtggctggatacgtcagtaccactttgactattggggccgaggcaccctggtcaccgtctcgagt

SEQ ID NO: 22 - protein, 123 aa, synthetic construct
  REGION 1..123: note = Homo sapiensIL330020 VH PRT
QVQLVQSGAEVKKPGASVKVSCKASGYTFTSYGISWVRQAPGQGLEWMGWISDYQGYTKYAEKFQGRVTMTTDTSTNTAYMELRSLRSDDTAVYYCARLYSSGWIRQYHFDYWGRGTLVTVSS

SEQ ID NO: 23 - protein, 5 aa, synthetic construct
  REGION 1..5: note = Homo sapiensIL330020 VH CDR1 PRT
SYGIS

SEQ ID NO: 24 - protein, 17 aa, synthetic construct
  REGION 1..17: note = Homo sapiensIL330020 VH CDR2 PRT
WISDYQGYTKYAEKFQG

SEQ ID NO: 25 - protein, 14 aa, synthetic construct
  REGION 1..14: note = Homo sapiensIL330020 VH CDR3 PRT
LYSSGWIRQYHFDY

SEQ ID NO: 26 - DNA, 315 bp, synthetic construct
  misc_feature 1..315: note = Homo sapiensIL330020 VL DNA
  source 1..315: mol_type = other DNA
tcctatgagctgactcagccaccctcagtgtccgtgtccccaggacagacagccagcatcacctgctcaggagataatttgaaagataaatatgtctcatggtatcagcagaagccagggcaggcccctgtactggttctctatcaagatagaaagcggccctcagggatccctgagcgattctctggctccaactcagggaacacagccactctgaccatcagcgggacccaggctatggatgaggctgactattattgtcaggcgtgggacagcggcactgccttcggcggagggaccaaggtcaccgtccta

SEQ ID NO: 27 - protein, 105 aa, synthetic construct
  REGION 1..105: note = Homo sapiensIL330020 VL PRT
SYELTQPPSVSVSPGQTASITCSGDNLKDKYVSWYQQKPGQAPVLVLYQDRKRPSGIPERFSGSNSGNTATLTISGTQAMDEADYYCQAWDSGTAFGGGTKVTVL

SEQ ID NO: 28 - protein, 11 aa, synthetic construct
  REGION 1..11: note = Homo sapiensIL330020 VL CDR1 PRT
SGDNLKDKYVS

SEQ ID NO: 29 - protein, 7 aa, synthetic construct
  REGION 1..7: note = Homo sapiensIL330020 VL CDR2 PRT
QDRKRPS

SEQ ID NO: 30 - protein, 8 aa, synthetic construct
  REGION 1..8: note = Homo sapiensIL330020 VL CDR3 PRT
QAWDSGTA

SEQ ID NO: 31 - DNA, 357 bp, synthetic construct
  misc_feature 1..357: note = Homo sapiensIL330071 VH DNA
  source 1..357: mol_type = other DNA
gaggtgcagctggtggagtctggagctgaggtgaagcagcctggggcctcagtgaaggtctcctgcaaggcttctggttacacctttaccagctatggtatcagctgggtgcgacaggcccctggacaagggcttgagtggatgggatggatcagcgcttacaatggtaacacaaactatgcacagaagctccagggcagagtcaccatgaccacagacacatccacgagcacagcctacatggagctgaggagcctgagatctgacgacacggccgtgtattactgtgcgagaaggggtttctatcatgatgcttttgatatctgggggcgagggaccacggtcaccgtctcgagt

SEQ ID NO: 32 - protein, 119 aa, synthetic construct
  REGION 1..119: note = Homo sapiensIL330071 VH PRT
EVQLVESGAEVKQPGASVKVSCKASGYTFTSYGISWVRQAPGQGLEWMGWISAYNGNTNYAQKLQGRVTMTTDTSTSTAYMELRSLRSDDTAVYYCARRGFYHDAFDIWGRGTTVTVSS

SEQ ID NO: 33 - protein, 5 aa, synthetic construct
  REGION 1..5: note = Homo sapiensIL330071 VH CDR1 PRT
SYGIS

SEQ ID NO: 34 - protein, 17 aa, synthetic construct
  REGION 1..17: note = Homo sapiensIL330071 VH CDR2 PRT
WISAYNGNTNYAQKLQG

SEQ ID NO: 35 - protein, 10 aa, synthetic construct
  REGION 1..10: note = Homo sapiensIL330071 VH CDR3 PRT
RGFYHDAFDI

SEQ ID NO: 36 - DNA, 321 bp, synthetic construct
  misc_feature 1..321: note = Homo sapiensIL330071 VL DNA
  source 1..321: mol_type = other DNA
gccatccagttgacccagtctccatcctccctgtctgcatctgtaggagacagagtcaccatcacttgccgggcgagtcagggcattagcaattatttagcctggtatcagcagaaaccagggaaagttcctaagctcctgatctatgctgcatccactttgcaatcaggggtcccatctcggttcagcggcagtggatctgggacagaattcactctcaccatcagcagcctgcagcctgatgattttgcaacttattactgccaacagtataatagttattctgtgacgttcggccaagggaccaaggtggaaatcaaa

SEQ ID NO: 37 - protein, 107 aa, synthetic construct
  REGION 1..107: note = Homo sapiensIL330071 VL PRT
AIQLTQSPSSLSASVGDRVTITCRASQGISNYLAWYQQKPGKVPKLLIYAASTLQSGVPSRFSGSGSGTEFTLTISSLQPDDFATYYCQQYNSYSVTFGQGTKVEIK

SEQ ID NO: 38 - protein, 11 aa, synthetic construct
  REGION 1..11: note = Homo sapiensIL330071 VL CDR1 PRT
RASQGISNYLA

SEQ ID NO: 39 - protein, 7 aa, synthetic construct
  REGION 1..7: note = Homo sapiensIL330071 VL CDR2 PRT
AASTLQS

SEQ ID NO: 40 - protein, 9 aa, synthetic construct
  REGION 1..9: note = Homo sapiensIL330071 VL CDR3 PRT
QQYNSYSVT

SEQ ID NO: 41 - DNA, 366 bp, synthetic construct
  misc_feature 1..366: note = Homo sapiensIL330125 VH DNA
  source 1..366: mol_type = other DNA
gaagtgcagctggtgcagtctggggctgaggtgaagaagcctggggcctcagtgactgtctcctgcaaggcttctggatacagcttcaccgactactatatacactgggtgcgacaggcccctggacaaggtcctgagtggatgggatggatcaaccctaacagtggtgtcacagactttgcgcagaagtttctgggcagggtcaccatgaccagggacacgtccatcagcacagcctacatggagctgagcagactgacatctgacgacacggccttgtattattgtgcgagagttgcctttgtatactatgatagtagtgccttccaatactggggcaaaggaaccctggtcaccgtctcgagt

SEQ ID NO: 42 - protein, 122 aa, synthetic construct
  REGION 1..122: note = Homo sapiensIL330125 VH PRT
EVQLVQSGAEVKKPGASVTVSCKASGYSFTDYYIHWVRQAPGQGPEWMGWINPNSGVTDFAQKFLGRVTMTRDTSISTAYMELSRLTSDDTALYYCARVAFVYYDSSAFQYWGKGTLVTVSS

SEQ ID NO: 43 - protein, 5 aa, synthetic construct
  REGION 1..5: note = Homo sapiensIL330125 VH CDR1 PRT
DYYIH

SEQ ID NO: 44 - protein, 17 aa, synthetic construct
  REGION 1..17: note = Homo sapiensIL330125 VH CDR2 PRT
WINPNSGVTDFAQKFLG

SEQ ID NO: 45 - protein, 13 aa, synthetic construct
  REGION 1..13: note = Homo sapiensIL330125 VH CDR3 PRT
VAFVYYDSSAFQY

SEQ ID NO: 46 - DNA, 324 bp, synthetic construct
  misc_feature 1..324: note = Homo sapiensIL330125 VL DNA
  source 1..324: mol_type = other DNA
ctgcctgtgctgactcagccaccctcagtgtccgtttccccaggacagacagccaccatcacctgctctgcagataagttgggggataaatatgctgcctggtatcagcagaagccaggccagtcccctgtcctggtcatctatcaagataggaagcggccctcagggatccctgagcgattctctggctccaactctgggaacacagccactctgatcatcagcgggacccaggctatggatgaggctgactattactgtcaggcgtgggacagcaacactggcctttatgtcttcggaactgggaccaagctgaccgtccta

SEQ ID NO: 47 - protein, 108 aa, synthetic construct
  REGION 1..108: note = Homo sapiensIL330125 VL PRT
LPVLTQPPSVSVSPGQTATITCSADKLGDKYAAWYQQKPGQSPVLVIYQDRKRPSGIPERFSGSNSGNTATLIISGTQAMDEADYYCQAWDSNTGLYVFGTGTKLTVL

SEQ ID NO: 48 - protein, 11 aa, synthetic construct
  REGION 1..11: note = Homo sapiensIL330125 VL CDR1 PRT
SADKLGDKYAA

SEQ ID NO: 49 - protein, 7 aa, synthetic construct
  REGION 1..7: note = Homo sapiensIL330125 VL CDR2 PRT
QDRKRPS

SEQ ID NO: 50 - protein, 11 aa, synthetic construct
  REGION 1..11: note = Homo sapiensIL330125 VL CDR3 PRT
QAWDSNTGLYV

SEQ ID NO: 51 - DNA, 378 bp, synthetic construct
  misc_feature 1..378: note = Homo sapiensIL330126 VH DNA
  source 1..378: mol_type = other DNA
gaggtccagctggtacagtctggggctgaactgaagaagcctggggcctcagtgaaggtctcctgcaagacttctggttacagttttaacacctatggtatcagttgggtgcgacaggcccctggacaagggcttgagtggatgggatgggtcagtggtgacgatggtaacataaattatgcagagaagttccagggcagagtcgccatgaccacagacacatccacgaccacagcctacatggagctgtggagcctgacatctgacgacacggccgtctattactgtgcgagagtacgtcgaggcagtggctggtacaagaactatcactactacatggacgtctggggccaagggacaatggtcaccgtctcgagt

SEQ ID NO: 52 - protein, 126 aa, synthetic construct
  REGION 1..126: note = Homo sapiensIL330126 VH PRT
EVQLVQSGAELKKPGASVKVSCKTSGYSFNTYGISWVRQAPGQGLEWMGWVSGDDGNINYAEKFQGRVAMTTDTSTTTAYMELWSLTSDDTAVYYCARVRRGSGWYKNYHYYMDVWGQGTMVTVSS

SEQ ID NO: 53 - protein, 5 aa, synthetic construct
  REGION 1..5: note = Homo sapiensIL330126 VH CDR1 PRT
TYGIS

SEQ ID NO: 54 - protein, 17 aa, synthetic construct
  REGION 1..17: note = Homo sapiensIL330126 VH CDR2 PRT
WVSGDDGNINYAEKFQG

SEQ ID NO: 55 - protein, 17 aa, synthetic construct
  REGION 1..17: note = Homo sapiensIL330126 VH CDR3 PRT
VRRGSGWYKNYHYYMDV

SEQ ID NO: 56 - DNA, 318 bp, synthetic construct
  misc_feature 1..318: note = Homo sapiensIL330126 VL DNA
  source 1..318: mol_type = other DNA
cagtctgtgctgactcagccaccctcagtgtccgtgtccccaggacagacagccagcgtcacctgctctggagatagattgggggataaatatgcttcctggtatcagcagaagccaggccagtcccctgtcttggtcatctatcaagataggaagcggccctcagggatccctgagcgattctctggctccaactctgggaacacagccactctgaccatcagcgggacccaggctatggatgaggctgactattattgtcaggcgtgggacggcagtactgcgctattcggcggagggaccaagctgaccgtccta

SEQ ID NO: 57 - protein, 106 aa, synthetic construct
  REGION 1..106: note = Homo sapiensIL330126 VL PRT
QSVLTQPPSVSVSPGQTASVTCSGDRLGDKYASWYQQKPGQSPVLVIYQDRKRPSGIPERFSGSNSGNTATLTISGTQAMDEADYYCQAWDGSTALFGGGTKLTVL

SEQ ID NO: 58 - protein, 11 aa, synthetic construct
  REGION 1..11: note = Homo sapiensIL330126 VL CDR1 PRT
SGDRLGDKYAS

SEQ ID NO: 59 - protein, 7 aa, synthetic construct
  REGION 1..7: note = Homo sapiensIL330126 VL CDR2 PRT
QDRKRPS

SEQ ID NO: 60 - protein, 9 aa, synthetic construct
  REGION 1..9: note = Homo sapiensIL330126 VL CDR3 PRT
QAWDGSTAL

SEQ ID NO: 61 - DNA, 366 bp, synthetic construct
  misc_feature 1..366: note = Homo sapiensIL330425 VH DNA
  source 1..366: mol_type = other DNA
caggtgcagctggtgcagtctgggggaggcgtggtccagcctgggaggtccctgagactctcctgtgcagcctctggattcaccttcagtgaatatagtatgcactgggtccgccaggctccagggaagggactggaatatgtttcaactattagtagtaatggggctggcacatactacgcagactccgtgaagggcagagtcaccatctccagagacaattccaagaacacgctgtatgttcaaatgagcagtctgagacctgaggacacggctgtctattactgtgtgaaatccctaactaaatacccctatggtaactactttgactactggggcagagggaccacggtcaccgtctcctca

SEQ ID NO: 62 - protein, 122 aa, synthetic construct
  REGION 1..122: note = Homo sapiensIL330425 VH PRT
QVQLVQSGGGVVQPGRSLRLSCAASGFTFSEYSMHWVRQAPGKGLEYVSTISSNGAGTYYADSVKGRVTISRDNSKNTLYVQMSSLRPEDTAVYYCVKSLTKYPYGNYFDYWGRGTTVTVSS

SEQ ID NO: 63 - protein, 5 aa, synthetic construct
  REGION 1..5: note = Homo sapiensIL330425 VH CDR1 PRT
EYSMH

SEQ ID NO: 64 - protein, 17 aa, synthetic construct
  REGION 1..17: note = Homo sapiensIL330425 VH CDR2 PRT
TISSNGAGTYYADSVKG

SEQ ID NO: 65 - protein, 13 aa, synthetic construct
  REGION 1..13: note = Homo sapiensIL330425 VH CDR3 PRT
SLTKYPYGNYFDY

SEQ ID NO: 66 - DNA, 324 bp, synthetic construct
  misc_feature 1..324: note = Homo sapiensIL330425 VL DNA
  source 1..324: mol_type = other DNA
tcgtctgagctgactcaggaccctgctgtgtctgtggccttgggacagacagtcaggatcacatgccaaggagacagcctcagaagctattatgcaagctggtaccagcagaagccaggacaggcccctgtacttgtcatctatggtaaaaacaaccggccctcagggatcccagaccgattctctggctccagctcaggaaacacagcttccttgaccatcactagggctcaggcggaagatgaggctgactattactgtaactcccgggacagcagtggtaaccatgtggtattcggcggagggaccaagctgaccgtccta

SEQ ID NO: 67 - protein, 108 aa, synthetic construct
  REGION 1..108: note = Homo sapiensIL330425 VL PRT
SSELTQDPAVSVALGQTVRITCQGDSLRSYYASWYQQKPGQAPVLVIYGKNNRPSGIPDRFSGSSSGNTASLTITRAQAEDEADYYCNSRDSSGNHVVFGGGTKLTVL

SEQ ID NO: 68 - protein, 11 aa, synthetic construct
  REGION 1..11: note = Homo sapiensIL330425 VL CDR1 PRT
QGDSLRSYYAS

SEQ ID NO: 69 - protein, 7 aa, synthetic construct
  REGION 1..7: note = Homo sapiensIL330425 VL CDR2 PRT
GKNNRPS

SEQ ID NO: 70 - protein, 11 aa, synthetic construct
  REGION 1..11: note = Homo sapiensIL330425 VL CDR3 PRT
NSRDSSGNHVV

SEQ ID NO: 71 - DNA, 375 bp, synthetic construct
  misc_feature 1..375: note = Homo sapiensIL330428 VH DNA
  source 1..375: mol_type = other DNA
caggtgcagctggtgcaatctggggctgagacgaagaagtctggggcctcagtgaaggtctcttgcaagacttctggttacacctttgataactttggtatcagttgggtgcgacaggcccctggacaagggctggagtggataggatggatcagcatttacaatggaaacacagattatgcacagaatcttcggggcagactcaccttgaccacagacacgtccacgagtacagtccacatggaactgaagagcctgagatctgacgacacggccatttattactgtgcgagaggagggggtattagcagcagctggacccctgactactactttgactactggggccagggcaccctggtcaccgtctcctca

SEQ ID NO: 72 - protein, 125 aa, synthetic construct
  REGION 1..125: note = Homo sapiensIL330428 VH PRT
QVQLVQSGAETKKSGASVKVSCKTSGYTFDNFGISWVRQAPGQGLEWIGWISIYNGNTDYAQNLRGRLTLTTDTSTSTVHMELKSLRSDDTAIYYCARGGGISSSWTPDYYFDYWGQGTLVTVSS

SEQ ID NO: 73 - protein, 5 aa, synthetic construct
  REGION 1..5: note = Homo sapiensIL330428 VH CDR1 PRT
NFGIS

SEQ ID NO: 74 - protein, 17 aa, synthetic construct
  REGION 1..17: note = Homo sapiensIL330428 VH CDR2 PRT
WISIYNGNTDYAQNLRG

SEQ ID NO: 75 - protein, 16 aa, synthetic construct
  REGION 1..16: note = Homo sapiensIL330428 VH CDR3 PRT
GGGISSSWTPDYYFDY

SEQ ID NO: 76 - DNA, 324 bp, synthetic construct
  misc_feature 1..324: note = Homo sapiensIL330428 VL DNA
  source 1..324: mol_type = other DNA
tcgtctgagctgactcaggaccctgctgtgtctgtggcctcgggacagacagtccgtctcacatgccaaggagacactctcagaaattattattcaaactggtaccaacagaggccaggacaggcccccgttcttgtcctctacgggaacaacaggcggcccccgggaatcccagctcgattctctggctcccactcaggaaacacaggttccctgatcatcactggggctcaggcggaagatgaggctgagtatcactgtgccgcccgggatagcagtggcgaccatgttgtcttcggtggtgggaccaaggtcaccgtccta

SEQ ID NO: 77 - protein, 108 aa, synthetic construct
  REGION 1..108: note = Homo sapiensIL330428 VL PRT
SSELTQDPAVSVASGQTVRLTCQGDTLRNYYSNWYQQRPGQAPVLVLYGNNRRPPGIPARFSGSHSGNTGSLIITGAQAEDEAEYHCAARDSSGDHVVFGGGTKVTVL

SEQ ID NO: 78 - protein, 11 aa, synthetic construct
  REGION 1..11: note = Homo sapiensIL330428 VL CDR1 PRT
QGDTLRNYYSN

SEQ ID NO: 79 - protein, 7 aa, synthetic construct
  REGION 1..7: note = Homo sapiensIL330428 VL CDR2 PRT
GNNRRPP

SEQ ID NO: 80 - protein, 11 aa, synthetic construct
  REGION 1..11: note = Homo sapiensIL330428 VL CDR3 PRT
AARDSSGDHVV

SEQ ID NO: 81 - DNA, 339 bp, synthetic construct
  misc_feature 1..339: note = Homo sapiensIL330065 VH DNA
  source 1..339: mol_type = other DNA
gaggtccagctggtgcagtctggggctgaggtgaagaagcctgggactgcagtgaagatctcctgcaaggcttctggatacaccttcaccgactactacattcattgggtccaacaggcccctggaaaagggcttgagtggatgggacttgttgatcctgaagacggtgaaacaaaatacgcagagaaattccagggccgagtctccataaccgcggacacgtcgactgacacagcctacatggagctgaggagcctgacatctgaggacacggccgtgtatttctgcacaatggggtgggctcagtggggccgaggaaccctggtcaccgtctcgagt

SEQ ID NO: 82 - protein, 113 aa, synthetic construct
  REGION 1..113: note = Homo sapiensIL330065 VH PRT
EVQLVQSGAEVKKPGTAVKISCKASGYTFTDYYIHWVQQAPGKGLEWMGLVDPEDGETKYAEKFQGRVSITADTSTDTAYMELRSLTSEDTAVYFCTMGWAQWGRGTLVTVSS

SEQ ID NO: 83 - protein, 5 aa, synthetic construct
  REGION 1..5: note = Homo sapiensIL330065 VH CDR1 PRT
DYYIH

SEQ ID NO: 84 - protein, 17 aa, synthetic construct
  REGION 1..17: note = Homo sapiensIL330065 VH CDR2 PRT
LVDPEDGETKYAEKFQG

SEQ ID NO: 85 - protein, 4 aa, synthetic construct
  REGION 1..4: note = Homo sapiensIL330065 VH CDR3 PRT
GWAQ

SEQ ID NO: 86 - DNA, 330 bp, synthetic construct
  misc_feature 1..330: note = Homo sapiensIL330065 VL DNA
  source 1..330: mol_type = other DNA
cagtctgtgttgacgcagccgccctcagcgtctgggacccccgggcagagggtcaccatctcttgttctggaagcagctccaacatcggaagtaattatgtatactggtaccagcaggtcccaggaacggcccccaaactcgtcatctatagggattttcagcggccctcaggggtccctgaccgattttccggctccaagtctggcaactcagcctccctggtcatcagtggcctccggtccgaggatgagggtgaatatgtctgtgcagcatgggatgacagcctgactggtccaagattcggcggagggaccaaggtcaccgtccta

SEQ ID NO: 87 - protein, 110 aa, synthetic construct
  REGION 1..110: note = Homo sapiensIL330065 VL PRT
QSVLTQPPSASGTPGQRVTISCSGSSSNIGSNYVYWYQQVPGTAPKLVIYRDFQRPSGVPDRFSGSKSGNSASLVISGLRSEDEGEYVCAAWDDSLTGPRFGGGTKVTVL

SEQ ID NO: 88 - protein, 13 aa, synthetic construct
  REGION 1..13: note = Homo sapiensIL330065 VL CDR1 PRT
SGSSSNIGSNYVY

SEQ ID NO: 89 - protein, 7 aa, synthetic construct
  REGION 1..7: note = Homo sapiensIL330065 VL CDR2 PRT
RDFQRPS

SEQ ID NO: 90 - protein, 11 aa, synthetic construct
  REGION 1..11: note = Homo sapiensIL330065 VL CDR3 PRT
AAWDDSLTGPR

SEQ ID NO: 91 - DNA, 393 bp, synthetic construct
  misc_feature 1..393: note = Homo sapiensIL330099 VH DNA
  source 1..393: mol_type = other DNA
caggtacagctgcagcagtcaggggctgaggtgaagaagcctggggcctcagtgaaggtttcctgcaaggcatctggatacaccttcaccagcttctatatgaactgggtgcgacaggcccccggacaagggcttgagtggatgggaataatcagccctcgtggtggtacgacaagttacgcacagaacttccagggcagagtcaccatgaccagggacacgtccacaagcacagtctacatggagctgagtggcctgagatctgacgacacggccgtctattactgtgcgacagagtccttttactatgggtcggggacttattctggcgattattacctctactccggtatggccgactggggcaaaggaaccctggtcaccgtctcctca

SEQ ID NO: 92 - protein, 131 aa, synthetic construct
  REGION 1..131: note = Homo sapiensIL330099 VH PRT
QVQLQQSGAEVKKPGASVKVSCKASGYTFTSFYMNWVRQAPGQGLEWMGIISPRGGTTSYAQNFQGRVTMTRDTSTSTVYMELSGLRSDDTAVYYCATESFYYGSGTYSGDYYLYSGMADWGKGTLVTVSS

SEQ ID NO: 93 - protein, 5 aa, synthetic construct
  REGION 1..5: note = Homo sapiensIL330099 VH CDR1 PRT
SFYMN

SEQ ID NO: 94 - protein, 17 aa, synthetic construct
  REGION 1..17: note = Homo sapiensIL330099 VH CDR2 PRT
IISPRGGTTSYAQNFQG

SEQ ID NO: 95 - protein, 22 aa, synthetic construct
  REGION 1..22: note = Homo sapiensIL330099 VH CDR3 PRT
ESFYYGSGTYSGDYYLYSGMAD

SEQ ID NO: 96 - DNA, 324 bp, synthetic construct
  misc_feature 1..324: note = Homo sapiensIL330099 VL DNA
  source 1..324: mol_type = other DNA
tcgtctgagctgactcaggaccctgctgtgtctgcggccttgggacagacagtcaggatcacatgccaaggagacagcctcagaagctattatgcaagctggtaccagcagaagccaggacaggcccctgtacttgtcatctatggtaaaaacgaccggccctcagggatcccagaccgattctctggctccagctcaggaaacacagcttccttgaccatcactggggctcaggcggaagatgaggctgactattactgtaactcccgggacagcagtggtaaccatgtggtattcggcggagggaccaagctgaccgtccta

SEQ ID NO: 97 - protein, 108 aa, synthetic construct
  REGION 1..108: note = Homo sapiensIL330099 VL PRT
SSELTQDPAVSAALGQTVRITCQGDSLRSYYASWYQQKPGQAPVLVIYGKNDRPSGIPDRFSGSSSGNTASLTITGAQAEDEADYYCNSRDSSGNHVVFGGGTKLTVL

SEQ ID NO: 98 - protein, 11 aa, synthetic construct
  REGION 1..11: note = Homo sapiensIL330099 VL CDR1 PRT
QGDSLRSYYAS

SEQ ID NO: 99 - protein, 7 aa, synthetic construct
  REGION 1..7: note = Homo sapiensIL330099 VL CDR2 PRT
GKNDRPS

SEQ ID NO: 100 - protein, 11 aa, synthetic construct
  REGION 1..11: note = Homo sapiensIL330099 VL CDR3 PRT
NSRDSSGNHVV

SEQ ID NO: 101 - DNA, 351 bp, synthetic construct
  misc_feature 1..351: note = Homo sapiensIL330101 VH DNA
  source 1..351: mol_type = other DNA
gaggtgcagctgttggagtctgggggaggcttggtacagcctggggggtccctgagactctcctgtgcagcctctggattcacctttagcagctatgccatgagctgggtccgccaggctccagggaaggggctggagtgggtctcagctattagtggtagtggtggtagcacatactacgcagactccgtgaagggccggttcaccatctccagagacaattccaagaacacgctgtatctgcaaatgaacagcctgagagccgaggacacggccgtgtattactgtgtgagagtggtggctggctactttgactcctggggccggggaaccctggtcaccgtctcgagt

SEQ ID NO: 102 - protein, 117 aa, synthetic construct
  REGION 1..117: note = Homo sapiensIL330101 VH PRT
EVQLLESGGGLVQPGGSLRLSCAASGFTFSSYAMSWVRQAPGKGLEWVSAISGSGGSTYYADSVKGRFTISRDNSKNTLYLQMNSLRAEDTAVYYCVRVVAGYFDSWGRGTLVTVSS

SEQ ID NO: 103 - protein, 5 aa, synthetic construct
  REGION 1..5: note = Homo sapiensIL330101 VH CDR1 PRT
SYAMS

SEQ ID NO: 104 - protein, 17 aa, synthetic construct
  REGION 1..17: note = Homo sapiensIL330101 VH CDR2 PRT
AISGSGGSTYYADSVKG

SEQ ID NO: 105 - protein, 8 aa, synthetic construct
  REGION 1..8: note = Homo sapiensIL330101 VH CDR3 PRT
VVAGYFDS

SEQ ID NO: 106 - DNA, 324 bp, synthetic construct
  misc_feature 1..324: note = Homo sapiensIL330101 VL DNA
  source 1..324: mol_type = other DNA
tcctatgtgctgactcagccaccctcggtgtcagtgtccccaggacagacggccaggatcacctgctctggcgatgctttgccaaagcaatatgctcattggtaccagcagaagccaggccaggcccctgcactggtgatatataaagacactgagaggccctcagggattcctgagcgattctctgggtccagctcagggacaacagtcacgctgaccatcagtggagtccaggcagaagatgaagctgactattactgtcaatcagcagacagtagtggtgcttcacgggtgttcggcggagggaccaaggtcaccgtccta

SEQ ID NO: 107 - protein, 108 aa, synthetic construct
  REGION 1..108: note = Homo sapiensIL330101 VL PRT
SYVLTQPPSVSVSPGQTARITCSGDALPKQYAHWYQQKPGQAPALVIYKDTERPSGIPERFSGSSSGTTVTLTISGVQAEDEADYYCQSADSSGASRVFGGGTKVTVL

SEQ ID NO: 108 - protein, 11 aa, synthetic construct
  REGION 1..11: note = Homo sapiensIL330101 VL CDR1 PRT
SGDALPKQYAH

SEQ ID NO: 109 - protein, 7 aa, synthetic construct
  REGION 1..7: note = Homo sapiensIL330101 VL CDR2 PRT
KDTERPS

SEQ ID NO: 110 - protein, 11 aa, synthetic construct
  REGION 1..11: note = Homo sapiensIL330101 VL CDR3 PRT
QSADSSGASRV

SEQ ID NO: 111 - DNA, 351 bp, synthetic construct; identical to SEQ ID NO: 101
  misc_feature 1..351: note = Homo sapiensIL330101_fgl VH DNA
  source 1..351: mol_type = other DNA

SEQ ID NO: 112 - protein, 117 aa, synthetic construct; identical to SEQ ID NO: 102
  REGION 1..117: note = Homo sapiensIL330101_fgl VH PRT

SEQ ID NO: 113 - protein, 5 aa, synthetic construct
  REGION 1..5: note = Homo sapiensIL330101_fgl VH CDR1 PRT
SYAMS

SEQ ID NO: 114 - protein, 17 aa, synthetic construct
  REGION 1..17: note = Homo sapiensIL330101_fgl VH CDR2 PRT
AISGSGGSTYYADSVKG

SEQ ID NO: 115 - protein, 8 aa, synthetic construct
  REGION 1..8: note = Homo sapiensIL330101_fgl VH CDR3 PRT
VVAGYFDS

SEQ ID NO: 116 - DNA, 324 bp, synthetic construct
  misc_feature 1..324: note = Homo sapiensIL330101_fgl VL DNA
  source 1..324: mol_type = other DNA
tcctatgagctgatgcagccaccctcggtgtcagtgtccccaggacagacggccaggatcacctgctctggcgatgctttgccaaagcaatatgctcattggtaccagcagaagccaggccaggcccctgtgctggtgatatataaagacactgagaggccctcagggattcctgagcgattctctgggtccagctcagggacaacagtcacgctgaccatcagtggagtccaggcagaagatgaagctgactattactgtcaatcagcagacagtagtggtgcttcacgggtgttcggcggagggaccaagctgaccgtccta

SEQ ID NO: 117 - protein, 108 aa, synthetic construct
  REGION 1..108: note = Homo sapiensIL330101_fgl VL PRT
SYELMQPPSVSVSPGQTARITCSGDALPKQYAHWYQQKPGQAPVLVIYKDTERPSGIPERFSGSSSGTTVTLTISGVQAEDEADYYCQSADSSGASRVFGGGTKLTVL

SEQ ID NO: 118 - protein, 11 aa, synthetic construct
  REGION 1..11: note = Homo sapiensIL330101_fgl VL CDR1 PRT
SGDALPKQYAH

SEQ ID NO: 119 - protein, 7 aa, synthetic construct
  REGION 1..7: note = Homo sapiensIL330101_fgl VL CDR2 PRT
KDTERPS

SEQ ID NO: 120 - protein, 11 aa, synthetic construct
  REGION 1..11: note = Homo sapiensIL330101_fgl VL CDR3 PRT
QSADSSGASRV

SEQ ID NO: 121 - DNA, 357 bp, synthetic construct
  misc_feature 1..357: note = Homo sapiensIL330107 VH DNA
  source 1..357: mol_type = other DNA
cagatgcagctggtgcagtctgggggaggcgtggtccagcctggggggtccctgagactctcctgtgcagcctctggattcacctttagcagctatgccatgagctgggtccgccaggctccagggaaggggctggagtgggtctcagctattagtggtagtggtggtagcacatactacgcagactccgtgaagggccggttcaccatctccagagacaattccaagaacacgctgtatctgcaaatgaacagcctgagagccgaggacacggccgtatattactgtgcgaaaccgttccccagctactggtacttcgatctctggggcaaaggcaccctggtcaccgtctcgagt

SEQ ID NO: 122 - protein, 119 aa, synthetic construct
  REGION 1..119: note = Homo sapiensIL330107 VH PRT
QMQLVQSGGGVVQPGGSLRLSCAASGFTFSSYAMSWVRQAPGKGLEWVSAISGSGGSTYYADSVKGRFTISRDNSKNTLYLQMNSLRAEDTAVYYCAKPFPSYWYFDLWGKGTLVTVSS

SEQ ID NO: 123 - protein, 5 aa, synthetic construct
  REGION 1..5: note = Homo sapiensIL330107 VH CDR1 PRT
SYAMS

SEQ ID NO: 124 - protein, 17 aa, synthetic construct
  REGION 1..17: note = Homo sapiensIL330107 VH CDR2 PRT
AISGSGGSTYYADSVKG

SEQ ID NO: 125 - protein, 10 aa, synthetic construct
  REGION 1..10: note = Homo sapiensIL330107 VH CDR3 PRT
PFPSYWYFDL

SEQ ID NO: 126 - DNA, 324 bp, synthetic construct
  misc_feature 1..324: note = Homo sapiensIL330107 VL DNA
  source 1..324: mol_type = other DNA
tcctatgtgctgactcagccaccctcggtgtcagtgtccccaggacagacggccaggatcacctgctctggagatgcattgccaaagcaatatgcttattggtaccagcagaagccaggccaggcccctgtgctggtgatatataaagacagtgagaggccctcagggatccctgagcgattctctggctccagctcagggacaacagtcacgttgaccatcagtggagtccaggcagaagacgaggctgactattactgtcaatcagcagacagcagtggtacttatcgggtgttcggcggagggacccagctcaccgtttta

SEQ ID NO: 127 - protein, 108 aa, synthetic construct
  REGION 1..108: note = Homo sapiensIL330107 VL PRT
SYVLTQPPSVSVSPGQTARITCSGDALPKQYAYWYQQKPGQAPVLVIYKDSERPSGIPERFSGSSSGTTVTLTISGVQAEDEADYYCQSADSSGTYRVFGGGTQLTVL

SEQ ID NO: 128 - protein, 11 aa, synthetic construct
  REGION 1..11: note = Homo sapiensIL330107 VL CDR1 PRT
SGDALPKQYAY

SEQ ID NO: 129 - protein, 7 aa, synthetic construct
  REGION 1..7: note = Homo sapiensIL330107 VL CDR2 PRT
KDSERPS

SEQ ID NO: 130 - protein, 11 aa, synthetic construct
  REGION 1..11: note = Homo sapiensIL330107 VL CDR3 PRT
QSADSSGTYRV

SEQ ID NO: 131 - DNA, 363 bp, synthetic construct
  misc_feature 1..363: note = Homo sapiensIL330149 VH DNA
  source 1..363: mol_type = other DNA
gaggtgcagctgttggagtctgggggaggcttggtacagcctggggggtccctgagactctcctgtgcagcctctggattcacctttagcagctatgccatgagctgggtccgccaggctccagggaaggggctggagtgggtctcagctattagtggtagtggtggtagcacatactacgcagactccgtgaagggccggttcaccatctccagagacaattccaagaacacgctgtatctgcaaatgaacagcctgagagccgaggacacggccgtgtattactgtgtaagaaccttggcttacagcacgagctggttctttgactactggggcaggggaaccctggtcaccgtctcgagt

SEQ ID NO: 132 - protein, 121 aa, synthetic construct
  REGION 1..121: note = Homo sapiensIL330149 VH PRT
EVQLLESGGGLVQPGGSLRLSCAASGFTFSSYAMSWVRQAPGKGLEWVSAISGSGGSTYYADSVKGRFTISRDNSKNTLYLQMNSLRAEDTAVYYCVRTLAYSTSWFFDYWGRGTLVTVSS

SEQ ID NO: 133 - protein, 5 aa, synthetic construct
  REGION 1..5: note = Homo sapiensIL330149 VH CDR1 PRT
SYAMS

SEQ ID NO: 134 - protein, 17 aa, synthetic construct
  REGION 1..17: note = Homo sapiensIL330149 VH CDR2 PRT
AISGSGGSTYYADSVKG

SEQ ID NO: 135 - protein, 12 aa, synthetic construct
  REGION 1..12: note = Homo sapiensIL330149 VH CDR3 PRT
TLAYSTSWFFDY

SEQ ID NO: 136 - DNA, 318 bp, synthetic construct
  misc_feature 1..318: note = Homo sapiensIL330149 VL DNA
  source 1..318: mol_type = other DNA
tcctatgagctgactcagccacccgcggtgtcagtgtccccaggacaaacggccaggatcacctgctctggagatgcattgccaaaaaaatatgcttattggtaccagcagaagtcaggccaggcccctgtgctggtcatctatgaggacgccaaacgaccctccgggatccctgagagattctctggctccagctcagggacaatggccaccttgactgtaagtggggcccaggtggaggatgaagctgactactactgttactcaacagacagcagtggtcctgtattcggcggagggaccaagctgaccgtccta

SEQ ID NO: 137 - protein, 106 aa, synthetic construct
  REGION 1..106: note = Homo sapiensIL330149 VL PRT
SYELTQPPAVSVSPGQTARITCSGDALPKKYAYWYQQKSGQAPVLVIYEDAKRPSGIPERFSGSSSGTMATLTVSGAQVEDEADYYCYSTDSSGPVFGGGTKLTVL

SEQ ID NO: 138 - protein, 11 aa, synthetic construct
  REGION 1..11: note = Homo sapiensIL330149 VL CDR1 PRT
SGDALPKKYAY

SEQ ID NO: 139 - protein, 7 aa, synthetic construct
  REGION 1..7: note = Homo sapiensIL330149 VL CDR2 PRT
EDAKRPS

SEQ ID NO: 140 - protein, 9 aa, synthetic construct
  REGION 1..9: note = Homo sapiensIL330149 VL CDR3 PRT
YSTDSSGPV

SEQ ID NO: 141 - DNA, 345 bp, synthetic construct
  misc_feature 1..345: note = Homo sapiensIL330180 VH DNA
  source 1..345: mol_type = other DNA
caggtacagctgcagcagtcaggggctgaggtgaagaagcctggggcctcagtgaaggtctcctgcaaggcttctggatacaccttcaccggctactatatgcactgggtgcgacaggcccctggacaagggcttgagtggatgggatggatcaaccctaacagtggtggcacaaactatgcacagaagtttcagggcagagtcaccatgaccagggacacgtccatcagcacagcctacatggagctgagcaggctgagatctgacgacacggccgtgtattactgtgcgagacggaacgcttttgatatctggggcaagggaaccctggtcaccgtctcgagt

SEQ ID NO: 142 - protein, 115 aa, synthetic construct
  REGION 1..115: note = Homo sapiensIL330180 VH PRT
QVQLQQSGAEVKKPGASVKVSCKASGYTFTGYYMHWVRQAPGQGLEWMGWINPNSGGTNYAQKFQGRVTMTRDTSISTAYMELSRLRSDDTAVYYCARRNAFDIWGKGTLVTVSS

SEQ ID NO: 143 - protein, 5 aa, synthetic construct
  REGION 1..5: note = Homo sapiensIL330180 VH CDR1 PRT
GYYMH

SEQ ID NO: 144 - protein, 17 aa, synthetic construct
  REGION 1..17: note = Homo sapiensIL330180 VH CDR2 PRT
WINPNSGGTNYAQKFQG

SEQ ID NO: 145 - protein, 6 aa, synthetic construct
  REGION 1..6: note = Homo sapiensIL330180 VH CDR3 PRT
RNAFDI

SEQ ID NO: 146 - DNA, 330 bp, synthetic construct
  misc_feature 1..330: note = Homo sapiensIL330180 VL DNA
  source 1..330: mol_type = other DNA
cagcctgtgctgactcagccaccctcggtgtctgaagcccccaggcagagggtcaccatctcctgttctggaagcagctccaacatcggaaataatgctgtaaactggtaccagcagctcccaggaacggcccccaaactcctcatctataggaataatcagcggccctcaggggtccctgaccgattctctggctccaagtctggcacctcagcctccctggccatcagtgggctccggtccgaggatgaggctgattattactgtgcagcatgggatgacagcctgagtggttgggtgttcggcggagggaccaaggtcaacgtccta

SEQ ID NO: 147 - protein, 110 aa, synthetic construct
  REGION 1..110: note = Homo sapiensIL330180 VL PRT
QPVLTQPPSVSEAPRQRVTISCSGSSSNIGNNAVNWYQQLPGTAPKLLIYRNNQRPSGVPDRFSGSKSGTSASLAISGLRSEDEADYYCAAWDDSLSGWVFGGGTKVNVL

SEQ ID NO: 148 - protein, 13 aa, synthetic construct
  REGION 1..13: note = Homo sapiensIL330180 VL CDR1 PRT
SGSSSNIGNNAVN

SEQ ID NO: 149 - protein, 7 aa, synthetic construct
  REGION 1..7: note = Homo sapiensIL330180 VL CDR2 PRT
RNNQRPS

SEQ ID NO: 150 - protein, 11 aa, synthetic construct
  REGION 1..11: note = Homo sapiensIL330180 VL CDR3 PRT
AAWDDSLSGWV

SEQ ID NO: 151 - DNA, 351 bp, synthetic construct
  misc_feature 1..351: note = Homo sapiensIL330259 VH DNA
  source 1..351: mol_type = other DNA
gaggtgcagctgttggagtctgggggaggcttggtacagcctggggggtccctgagactctcctgtgcagcctctggattcacctttagcagctatgccatgagctgggtccgccaggctccagggaaggggctggagtgggtctcagcgagcaccccctggcagggtagcacatactacgcagactccgtgaagggccggttcaccatctccagagacaattccaagaacacgctgtatctgcaaatgaacagcctgagagccgaggacacggccgtgtattactgtgtgagagtggtggctggctactttgactcctggggccggggaaccctggtcaccgtctcgagt

SEQ ID NO: 152 - protein, 117 aa, synthetic construct
  REGION 1..117: note = Homo sapiensIL330259 VH PRT
EVQLLESGGGLVQPGGSLRLSCAASGFTFSSYAMSWVRQAPGKGLEWVSASTPWQGSTYYADSVKGRFTISRDNSKNTLYLQMNSLRAEDTAVYYCVRVVAGYFDSWGRGTLVTVSS

SEQ ID NO: 153 - protein, 5 aa, synthetic construct
  REGION 1..5: note = Homo sapiensIL330259 VH CDR1 PRT
SYAMS

SEQ ID NO: 154 - protein, 17 aa, synthetic construct
  REGION 1..17: note = Homo sapiensIL330259 VH CDR2 PRT
ASTPWQGSTYYADSVKG

SEQ ID NO: 155 - protein, 8 aa, synthetic construct
  REGION 1..8: note = Homo sapiensIL330259 VH CDR3 PRT
VVAGYFDS

SEQ ID NO: 156 - DNA, 324 bp, synthetic construct; identical to SEQ ID NO: 106
  misc_feature 1..324: note = Homo sapiensIL330259 VL DNA
  source 1..324: mol_type = other DNA

SEQ ID NO: 157 - protein, 108 aa, synthetic construct; identical to SEQ ID NO: 107
  REGION 1..108: note = Homo sapiensIL330259 VL PRT

SEQ ID NO: 158 - protein, 11 aa, synthetic construct
  REGION 1..11: note = Homo sapiensIL330259 VL CDR1 PRT
SGDALPKQYAH

SEQ ID NO: 159 - protein, 7 aa, synthetic construct
  REGION 1..7: note = Homo sapiensIL330259 VL CDR2 PRT
KDTERPS

SEQ ID NO: 160 - protein, 11 aa, synthetic construct
  REGION 1..11: note = Homo sapiensIL330259 VL CDR3 PRT
QSADSSGASRV

SEQ ID NO: 161 - DNA, 351 bp, synthetic construct; identical to SEQ ID NO: 151
  misc_feature 1..351: note = Homo sapiensIL330259_fgl VH DNA
  source 1..351: mol_type = other DNA

SEQ ID NO: 162 - protein, 117 aa, synthetic construct; identical to SEQ ID NO: 152
  REGION 1..117: note = Homo sapiensIL330259_fgl VH PRT

SEQ ID NO: 163 - protein, 5 aa, synthetic construct
  REGION 1..5: note = Homo sapiensIL330259_fgl VH CDR1 PRT
SYAMS

SEQ ID NO: 164 - protein, 17 aa, synthetic construct
  REGION 1..17: note = Homo sapiensIL330259_fgl VH CDR2 PRT
ASTPWQGSTYYADSVKG

SEQ ID NO: 165 - protein, 8 aa, synthetic construct
  REGION 1..8: note = Homo sapiensIL330259_fgl VH CDR3 PRT
VVAGYFDS

SEQ ID NO: 166 - DNA, 324 bp, synthetic construct; identical to SEQ ID NO: 116
  misc_feature 1..324: note = Homo sapiensIL330259_fgl VL DNA
  source 1..324: mol_type = other DNA

SEQ ID NO: 167 - protein, 108 aa, synthetic construct; identical to SEQ ID NO: 117
  REGION 1..108: note = Homo sapiensIL330259_fgl VL PRT

SEQ ID NO: 168 - protein, 11 aa, synthetic construct
  REGION 1..11: note = Homo sapiensIL330259_fgl VL CDR1 PRT
SGDALPKQYAH

SEQ ID NO: 169 - protein, 7 aa, synthetic construct
  REGION 1..7: note = Homo sapiensIL330259_fgl VL CDR2 PRT
KDTERPS

SEQ ID NO: 170 - protein, 11 aa, synthetic construct
  REGION 1..11: note = Homo sapiensIL330259_fgl VL CDR3 PRT
QSADSSGASRV

SEQ ID NO: 171 - DNA, 351 bp, synthetic construct
  misc_feature 1..351: note = Homo sapiensH338L293 VH DNA
  source 1..351: mol_type = other DNA
gaggtgcagctgttggagtctgggggaggcttggtacagcctggggggtccctgagactctcctgtgcagcctctggattcacctttagcagctatgccatgagctgggtccgccaggctccagggaaggggctggagtgggtctcagctattagtccccgggaggggtggcagtactacgcagactccgtgaagggccggttcaccatctccagagacaattccaagaacacgctgtatctgcaaatgaacagcctgagagccgaggacacggccgtgtattactgtgtgagagtggtggctggctactttgactcctggggccggggaaccctggtcaccgtctcgagt

SEQ ID NO: 172 - protein, 117 aa, synthetic construct
  REGION 1..117: note = Homo sapiensH338L293 VH PRT
EVQLLESGGGLVQPGGSLRLSCAASGFTFSSYAMSWVRQAPGKGLEWVSAISPREGWQYYADSVKGRFTISRDNSKNTLYLQMNSLRAEDTAVYYCVRVVAGYFDSWGRGTLVTVSS

SEQ ID NO: 173 - protein, 5 aa, synthetic construct
  REGION 1..5: note = Homo sapiensH338L293 VH CDR1 PRT
SYAMS

SEQ ID NO: 174 - protein, 17 aa, synthetic construct
  REGION 1..17: note = Homo sapiensH338L293 VH CDR2 PRT
AISPREGWQYYADSVKG

SEQ ID NO: 175 - protein, 8 aa, synthetic construct
  REGION 1..8: note = Homo sapiensH338L293 VH CDR3 PRT
VVAGYFDS

SEQ ID NO: 176 - DNA, 324 bp, synthetic construct
  misc_feature 1..324: note = Homo sapiensH338L293 VL DNA
  source 1..324: mol_type = other DNA
tcctatgtgctgactcagccaccctcggtgtcagtgtccccaggacagacggccaggatcacctgctctggcgatgctttgccaaagcaatatgctcattggtaccagcagaagccaggccaggcccctgcactggtgatatataaagacactgagaggccctcagggattcctgagcgattctctgggtccagctcagggacaacagtcacgctgaccatcagtggagtccaggcagaagatgaagctgactattactgtatgagcagcgaccccagcggtgcttcacgggtgttcggcggagggaccaaggtcaccgtccta

SEQ ID NO: 177 - protein, 108 aa, synthetic construct
  REGION 1..108: note = Homo sapiensH338L293 VL PRT
SYVLTQPPSVSVSPGQTARITCSGDALPKQYAHWYQQKPGQAPALVIYKDTERPSGIPERFSGSSSGTTVTLTISGVQAEDEADYYCMSSDPSGASRVFGGGTKVTVL

SEQ ID NO: 178 - protein, 11 aa, synthetic construct
  REGION 1..11: note = Homo sapiensH338L293 VL CDR1 PRT
SGDALPKQYAH

SEQ ID NO: 179 - protein, 7 aa, synthetic construct
  REGION 1..7: note = Homo sapiensH338L293 VL CDR2 PRT
KDTERPS

SEQ ID NO: 180 - protein, 11 aa, synthetic construct
  REGION 1..11: note = Homo sapiensH338L293 VL CDR3 PRT
MSSDPSGASRV

SEQ ID NO: 181 - DNA, 351 bp, synthetic construct
  misc_feature 1..351: note = Homo sapiensH338L293_fgl VH DNA
  source 1..351: mol_type = other DNA
gaggtgcagctgttggagtctgggggaggcttggtacagcctggggggtccctgagactctcctgtgcagcctctggattcacctttagcagctatgccatgagctgggtccgccaggctccagggaaggggctggagtgggtctcagctattagtccccgggaggggtggcagtactacgcagactccgtgaagggccggttcaccatctccagagacaattccaagaacacgctgtatctgcaaatgaacagcctgagagccgaggacacggccgtgtattactgtgtgagagtggtggctggctactttgactcctggggccggggcaccctggtcaccgtctcgagt

SEQ ID NO: 182 - protein, 117 aa, synthetic construct; identical to SEQ ID NO: 172
  REGION 1..117: note = Homo sapiensH338L293_fgl VH PRT

SEQ ID NO: 183 - protein, 5 aa, synthetic construct
  REGION 1..5: note = Homo sapiensH338L293_fgl VH CDR1 PRT
SYAMS

SEQ ID NO: 184 - protein, 17 aa, synthetic construct
  REGION 1..17: note = Homo sapiensH338L293_fgl VH CDR2 PRT
AISPREGWQYYADSVKG

SEQ ID NO: 185 - protein, 8 aa, synthetic construct
  REGION 1..8: note = Homo sapiensH338L293_fgl VH CDR3 PRT
VVAGYFDS

SEQ ID NO: 186 - DNA, 324 bp, synthetic construct
  misc_feature 1..324: note = Homo sapiensH338L293_fgl VL DNA
  source 1..324: mol_type = other DNA
tcctatgagctgatgcagccaccctcggtgtcagtgtccccaggacagacggccaggatcacctgctctggcgatgctttgccaaagcaatatgctcattggtaccagcagaagccaggccaggcccctgtgctggtgatatataaagacactgagaggccctcagggattcctgagcgattctctgggtccagctcagggacaacagtcacgctgaccatcagtggagtccaggcagaagatgaagctgactattactgtatgtcctcggacccgagcggtgcttcacgggtgttcggcggagggaccaagctgaccgtccta

SEQ ID NO: 187 - protein, 108 aa, synthetic construct
  REGION 1..108: note = Homo sapiensH338L293_fgl VL PRT
SYELMQPPSVSVSPGQTARITCSGDALPKQYAHWYQQKPGQAPVLVIYKDTERPSGIPERFSGSSSGTTVTLTISGVQAEDEADYYCMSSDPSGASRVFGGGTKLTVL

SEQ ID NO: 188 - protein, 11 aa, synthetic construct
  REGION 1..11: note = Homo sapiensH338L293_fgl VL CDR1 PRT
SGDALPKQYAH

SEQ ID NO: 189 - protein, 7 aa, synthetic construct
  REGION 1..7: note = Homo sapiensH338L293_fgl VL CDR2 PRT
KDTERPS

SEQ ID NO: 190 - protein, 11 aa, synthetic construct
  REGION 1..11: note = Homo sapiensH338L293_fgl VL CDR3 PRT
MSSDPSGASRV

SEQ ID NO: 191 - DNA, 351 bp, synthetic construct
  misc_feature 1..351: note = Homo sapiensIL330377 VH DNA
  source 1..351: mol_type = other DNA
gaggtgcagctgttggagtctgggggaggcttggtacagcctggggggtccctgagactctcctgtgcagcctctggattcacctttagcagctatgccatgagctgggtccgccaggctccagggaaggggctggagtgggtctcagcgtccgacatgctctacggtagcacatactacgcagactccgtgaagggccggttcaccatctccagagacaattccaagaacacgctgtatctgcaaatgaacagcctgagagccgaggacacggccgtgtattactgttcccagaacatcctgggctactttgactcctggggccggggaaccctggtcaccgtctcgagt

SEQ ID NO: 192 - protein, 117 aa, synthetic construct
  REGION 1..117: note = Homo sapiensIL330377 VH PRT
EVQLLESGGGLVQPGGSLRLSCAASGFTFSSYAMSWVRQAPGKGLEWVSASDMLYGSTYYADSVKGRFTISRDNSKNTLYLQMNSLRAEDTAVYYCSQNILGYFDSWGRGTLVTVSS

SEQ ID NO: 193 - protein, 5 aa, synthetic construct
  REGION 1..5: note = Homo sapiensIL330377 VH CDR1 PRT
SYAMS

SEQ ID NO: 194 - protein, 17 aa, synthetic construct
  REGION 1..17: note = Homo sapiensIL330377 VH CDR2 PRT
ASDMLYGSTYYADSVKG

SEQ ID NO: 195 - protein, 8 aa, synthetic construct
  REGION 1..8: note = Homo sapiensIL330377 VH CDR3 PRT
NILGYFDS

SEQ ID NO: 196 - DNA, 324 bp, synthetic construct
  misc_feature 1..324: note = Homo sapiensIL330377 VL DNA
  source 1..324: mol_type = other DNA
tcctatgtgctgactcagccaccctcggtgtcagtgtccccaggacagacggccaggatcacctgctctggcgatgctttgccaaagcaatatgctcattggtaccagcagaagccaggccaggcccctgcactggtgatatataaagacactgagaggccctcagggattcctgagcgattctctgggtccagctcagggacaacagtcacgctgaccatcagtggagtccaggcagaagatgaagctgactattactgtcaatcagcagacagtacggggtaccaccgggtgttcggcggagggaccaaggtcaccgtctta

SEQ ID NO: 197 - protein, 108 aa, synthetic construct
  REGION 1..108: note = Homo sapiensIL330377 VL PRT
SYVLTQPPSVSVSPGQTARITCSGDALPKQYAHWYQQKPGQAPALVIYKDTERPSGIPERFSGSSSGTTVTLTISGVQAEDEADYYCQSADSTGYHRVFGGGTKVTVL

SEQ ID NO: 198 - protein, 11 aa, synthetic construct
  REGION 1..11: note = Homo sapiensIL330377 VL CDR1 PRT
SGDALPKQYAH

SEQ ID NO: 199 - protein, 7 aa, synthetic construct
  REGION 1..7: note = Homo sapiensIL330377 VL CDR2 PRT
KDTERPS

SEQ ID NO: 200 - protein, 11 aa, synthetic construct
  REGION 1..11: note = Homo sapiensIL330377 VL CDR3 PRT
QSADSTGYHRV

SEQ ID NO: 201 - DNA, 351 bp, synthetic construct; identical to SEQ ID NO: 191
  misc_feature 1..351: note = Homo sapiensIL330377_fgl VH DNA
  source 1..351: mol_type = other DNA

SEQ ID NO: 202 - protein, 117 aa, synthetic construct; identical to SEQ ID NO: 192
  REGION 1..117: note = Homo sapiensIL330377_fgl VH PRT

SEQ ID NO: 203 - protein, 5 aa, synthetic construct
  REGION 1..5: note = Homo sapiensIL330377_fgl VH CDR1 PRT
SYAMS

SEQ ID NO: 204 - protein, 17 aa, synthetic construct
  REGION 1..17: note = Homo sapiensIL330377_fgl VH CDR2 PRT
ASDMLYGSTYYADSVKG

SEQ ID NO: 205 - protein, 8 aa, synthetic construct
  REGION 1..8: note = Homo sapiensIL330377_fgl VH CDR3 PRT
NILGYFDS

SEQ ID NO: 206 - DNA, 324 bp, synthetic construct
  misc_feature 1..324: note = Homo sapiensIL330377_fgl VL DNA
  source 1..324: mol_type = other DNA
tcctatgagctgatgcagccaccctcggtgtcagtgtccccaggacagacggccaggatcacctgctctggcgatgctttgccaaagcaatatgctcattggtaccagcagaagccaggccaggcccctgtgctggtgatatataaagacactgagaggccctcagggattcctgagcgattctctgggtccagctcagggacaacagtcacgctgaccatcagtggagtccaggcagaagatgaagctgactattactgtcaatcagcagacagtacggggtaccaccgggtgttcggcggagggaccaagctgaccgtccta

SEQ ID NO: 207 - protein, 108 aa, synthetic construct
  REGION 1..108: note = Homo sapiensIL330377_fgl VL PRT
SYELMQPPSVSVSPGQTARITCSGDALPKQYAHWYQQKPGQAPVLVIYKDTERPSGIPERFSGSSSGTTVTLTISGVQAEDEADYYCQSADSTGYHRVFGGGTKLTVL

SEQ ID NO: 208 - protein, 11 aa, synthetic construct
  REGION 1..11: note = Homo sapiensIL330377_fgl VL CDR1 PRT
SGDALPKQYAH

SEQ ID NO: 209 - protein, 7 aa, synthetic construct
  REGION 1..7: note = Homo sapiensIL330377_fgl VL CDR2 PRT
KDTERPS

SEQ ID NO: 210 - protein, 11 aa, synthetic construct
  REGION 1..11: note = Homo sapiensIL330377_fgl VL CDR3 PRT
QSADSTGYHRV

SEQ ID NO: 211 - DNA, 351 bp, synthetic construct
  misc_feature 1..351: note = Homo sapiensIL330388 VH DNA
  source 1..351: mol_type = other DNA
gaggtgcagctgttggagtctgggggaggcttggtacagcctggggggtccctgagactctcctgtgcagcctctggattcacctttagcagctatgccatgagctgggtccgccaggctccagggaaggggctggagtgggtctcagctagcaccccctggcaaggtagcacatactacgcagactccgtgaagggccggttcaccatctccagagacaattccaagaacacgctgtatctgcaaatgaacagcctgagagccgaggacacggccgtgtattactgtgtgagatggtactgggggtggatcgactcctggggccggggaaccctggtcaccgtctcgagt

SEQ ID NO: 212 - protein, 117 aa, synthetic construct
  REGION 1..117: note = Homo sapiensIL330388 VH PRT
EVQLLESGGGLVQPGGSLRLSCAASGFTFSSYAMSWVRQAPGKGLEWVSASTPWQGSTYYADSVKGRFTISRDNSKNTLYLQMNSLRAEDTAVYYCVRWYWGWIDSWGRGTLVTVSS

SEQ ID NO: 213 - protein, 5 aa, synthetic construct
  REGION 1..5: note = Homo sapiensIL330388 VH CDR1 PRT
SYAMS

SEQ ID NO: 214 - protein, 17 aa, synthetic construct
  REGION 1..17: note = Homo sapiensIL330388 VH CDR2 PRT
ASTPWQGSTYYADSVKG

SEQ ID NO: 215 - protein, 8 aa, synthetic construct
  REGION 1..8: note = Homo sapiensIL330388 VH CDR3 PRT
WYWGWIDS

SEQ ID NO: 216 - DNA, 324 bp, synthetic construct
  misc_feature 1..324: note = Homo sapiensIL330388 VL DNA
  source 1..324: mol_type = other DNA
tcctatgtgctgactcagccaccctcggtgtcagtgtccccaggacagacggccaggatcacctgctctggcgatgctttgccaaagcaatatgctcattggtaccagcagaagccaggccaggcccctgcactggtgatatataaagacactgagaggccctcagggattcctgagcgattctctgggtccagctcagggacaacagtcacgctgaccatcagtggagtccaggcagaagatgaagctgactattactgtatgtcctcggacccgagcggtgcttcacgggtgttcggcggagggaccaaggtcaccgtccta

SEQ ID NO: 217 - protein, 108 aa, synthetic construct; identical to SEQ ID NO: 177
  REGION 1..108: note = Homo sapiensIL330388 VL PRT

SEQ ID NO: 218 - protein, 11 aa, synthetic construct
  REGION 1..11: note = Homo sapiensIL330388 VL CDR1 PRT
SGDALPKQYAH

SEQ ID NO: 219 - protein, 7 aa, synthetic construct
  REGION 1..7: note = Homo sapiensIL330388 VL CDR2 PRT
KDTERPS

SEQ ID NO: 220 - protein, 11 aa, synthetic construct
  REGION 1..11: note = Homo sapiensIL330388 VL CDR3 PRT
MSSDPSGASRV

SEQ ID NO: 221 - DNA, 351 bp, synthetic construct
  misc_feature 1..351: note = Homo sapiensIL330388_fgl VH DNA
  source 1..351: mol_type = other DNA
gaggtgcagctgttggagtctgggggaggcttggtacagcctggggggtccctgagactctcctgtgcagcctctggattcacctttagcagctatgccatgagctgggtccgccaggctccagggaaggggctggagtgggtctcagctagcaccccctggcaaggtagcacatactacgcagactccgtgaagggccggttcaccatctccagagacaattccaagaacacgctgtatctgcaaatgaacagcctgagagccgaggacacggccgtgtattactgtgtgagatggtactgggggtggatcgactcctggggccggggaaccctggtcaccgtctcctca

SEQ ID NO: 222 - protein, 117 aa, synthetic construct; identical to SEQ ID NO: 212
  REGION 1..117: note = Homo sapiensIL330388_fgl VH PRT

SEQ ID NO: 223 - protein, 5 aa, synthetic construct
  REGION 1..5: note = Homo sapiensIL330388_fgl VH CDR1 PRT
SYAMS

SEQ ID NO: 224 - protein, 17 aa, synthetic construct
  REGION 1..17: note = Homo sapiensIL330388_fgl VH CDR2 PRT
ASTPWQGSTYYADSVKG

SEQ ID NO: 225 - protein, 8 aa, synthetic construct
  REGION 1..8: note = Homo sapiensIL330388_fgl VH CDR3 PRT
WYWGWIDS

SEQ ID NO: 226 - DNA, 324 bp, synthetic construct; identical to SEQ ID NO: 186
  misc_feature 1..324: note = Homo sapiensIL330388_fgl VL DNA
  source 1..324: mol_type = other DNA

SEQ ID NO: 227 - protein, 108 aa, synthetic construct; identical to SEQ ID NO: 187
  REGION 1..108: note = Homo sapiensIL330388_fgl VL PRT

SEQ ID NO: 228 - protein, 11 aa, synthetic construct
  REGION 1..11: note = Homo sapiensIL330388_fgl VL CDR1 PRT
SGDALPKQYAH

SEQ ID NO: 229 - protein, 7 aa, synthetic construct
  REGION 1..7: note = Homo sapiensIL330388_fgl VL CDR2 PRT
KDTERPS

SEQ ID NO: 230 - protein, 11 aa, synthetic construct
  REGION 1..11: note = Homo sapiensIL330388_fgl VL CDR3 PRT
MSSDPSGASRV

SEQ ID NO: 231 - DNA, 351 bp, synthetic construct; identical to SEQ ID NO: 211
  misc_feature 1..351: note = Homo sapiensIL330396 VH DNA
  source 1..351: mol_type = other DNA

SEQ ID NO: 232 - protein, 117 aa, synthetic construct; identical to SEQ ID NO: 212
  REGION 1..117: note = Homo sapiensIL330396 VH PRT

SEQ ID NO: 233 - protein, 5 aa, synthetic construct
  REGION 1..5: note = Homo sapiensIL330396 VH CDR1 PRT
SYAMS

SEQ ID NO: 234 - protein, 17 aa, synthetic construct
  REGION 1..17: note = Homo sapiensIL330396 VH CDR2 PRT
ASTPWQGSTYYADSVKG

SEQ ID NO: 235 - protein, 8 aa, synthetic construct
  REGION 1..8: note = Homo sapiensIL330396 VH CDR3 PRT
WYWGWIDS

SEQ ID NO: 236 - DNA, 324 bp, synthetic construct
  misc_feature 1..324: note = Homo sapiensIL330396 VL DNA
  source 1..324: mol_type = other DNA
tcctatgtgctgactcagccaccctcggtgtcagtgtccccaggacagacggccaggatcacctgctctggcgatgctttgccaaagcaatatgctcattggtaccagcagaagccaggccaggcccctgcactggtgatatataaagacactgagaggccctcagggattcctgagcgattctctgggtccagctcagggacaacagtcacgctgaccatcagtggagtccaggcagaagatgaagctgactattactgtatgagcagcgacgacacgggtgcttcacgggtgttcggcggagggaccaaggtcaccgtccta

SEQ ID NO: 237 - protein, 108 aa, synthetic construct
  REGION 1..108: note = Homo sapiensIL330396 VL PRT
SYVLTQPPSVSVSPGQTARITCSGDALPKQYAHWYQQKPGQAPALVIYKDTERPSGIPERFSGSSSGTTVTLTISGVQAEDEADYYCMSSDDTGASRVFGGGTKVTVL

SEQ ID NO: 238 - protein, 11 aa, synthetic construct
  REGION 1..11: note = Homo sapiensIL330396 VL CDR1 PRT
SGDALPKQYAH

SEQ ID NO: 239 - protein, 7 aa, synthetic construct
  REGION 1..7: note = Homo sapiensIL330396 VL CDR2 PRT
KDTERPS

SEQ ID NO: 240 - protein, 11 aa, synthetic construct
  REGION 1..11: note = Homo sapiensIL330396 VL CDR3 PRT
MSSDDTGASRV

SEQ ID NO: 241 - DNA, 351 bp, synthetic construct; identical to SEQ ID NO: 211
  misc_feature 1..351: note = Homo sapiensIL330396_fgl VH DNA
  source 1..351: mol_type = other DNA

SEQ ID NO: 242 - protein, 117 aa, synthetic construct; identical to SEQ ID NO: 212
  REGION 1..117: note = Homo sapiensIL330396_fgl VH PRT

SEQ ID NO: 243 - protein, 5 aa, synthetic construct
  REGION 1..5: note = Homo sapiensIL330396_fgl VH CDR1 PRT
SYAMS

SEQ ID NO: 244 - protein, 17 aa, synthetic construct
  REGION 1..17: note = Homo sapiensIL330396_fgl VH CDR2 PRT
ASTPWQGSTYYADSVKG

SEQ ID NO: 245 - protein, 8 aa, synthetic construct
  REGION 1..8: note = Homo sapiensIL330396_fgl VH CDR3 PRT
WYWGWIDS

SEQ ID NO: 246 - DNA, 324 bp, synthetic construct
  misc_feature 1..324: note = Homo sapiensIL330396_fgl VL DNA
  source 1..324: mol_type = other DNA
tcctatgagctgatgcagccaccctcggtgtcagtgtccccaggacagacggccaggatcacctgctctggcgatgctttgccaaagcaatatgctcattggtaccagcagaagccaggccaggcccctgtgctggtgatatataaagacactgagaggccctcagggattcctgagcgattctctgggtccagctcagggacaacagtcacgctgaccatcagtggagtccaggcagaagatgaagctgactattactgtatgagcagcgacgacacgggtgcttcacgggtgttcggcggagggaccaagctgaccgtccta

SEQ ID NO: 247 - protein, 108 aa, synthetic construct
  REGION 1..108: note = Homo sapiensIL330396_fgl VL PRT
SYELMQPPSVSVSPGQTARITCSGDALPKQYAHWYQQKPGQAPVLVIYKDTERPSGIPERFSGSSSGTTVTLTISGVQAEDEADYYCMSSDDTGASRVFGGGTKLTVL

SEQ ID NO: 248 - protein, 11 aa, synthetic construct
  REGION 1..11: note = Homo sapiensIL330396_fgl VL CDR1 PRT
SGDALPKQYAH

SEQ ID NO: 249 - protein, 7 aa, synthetic construct
  REGION 1..7: note = Homo sapiensIL330396_fgl VL CDR2 PRT
KDTERPS

SEQ ID NO: 250 - protein, 11 aa, synthetic construct
  REGION 1..11: note = Homo sapiensIL330396_fgl VL CDR3 PRT
MSSDDTGASRV

SEQ ID NO: 251 - DNA, 351 bp, synthetic construct; identical to SEQ ID NO: 211
  misc_feature 1..351: note = Homo sapiensIL330398 VH DNA
  source 1..351: mol_type = other DNA

SEQ ID NO: 252 - protein, 117 aa, synthetic construct; identical to SEQ ID NO: 212
  REGION 1..117: note = Homo sapiensIL330398 VH PRT

SEQ ID NO: 253 - protein, 5 aa, synthetic construct
  REGION 1..5: note = Homo sapiensIL330398 VH CDR1 PRT
SYAMS

SEQ ID NO: 254 - protein, 17 aa, synthetic construct
  REGION 1..17: note = Homo sapiensIL330398 VH CDR2 PRT
ASTPWQGSTYYADSVKG

SEQ ID NO: 255 - protein, 8 aa, synthetic construct
  REGION 1..8: note = Homo sapiensIL330398 VH CDR3 PRT
WYWGWIDS

SEQ ID NO: 256 - DNA, 324 bp, synthetic construct
  misc_feature 1..324: note = Homo sapiensIL330398 VL DNA
  source 1..324: mol_type = other DNA
tcctatgtgctgactcagccaccctcggtgtcagtgtccccaggacagacggccaggatcacctgctctggcgatgctttgccaaagcaatatgctcattggtaccagcagaagccaggccaggcccctgcactggtgatatataaagacactgagaggccctcagggattcctgagcgattctctgggtccagctcagggacaacagtcacgctgaccatcagtggagtccaggcagaagatgaagctgactattactgtttgtccagcgacgcctcgggtgcttcacgggtgttcggcggagggaccaaggtcaccgtccta

SEQ ID NO: 257 - protein, 108 aa, synthetic construct
  REGION 1..108: note = Homo sapiensIL330398 VL PRT
SYVLTQPPSVSVSPGQTARITCSGDALPKQYAHWYQQKPGQAPALVIYKDTERPSGIPERFSGSSSGTTVTLTISGVQAEDEADYYCLSSDASGASRVFGGGTKVTVL

SEQ ID NO: 258 - protein, 11 aa, synthetic construct
  REGION 1..11: note = Homo sapiensIL330398 VL CDR1 PRT
SGDALPKQYAH

SEQ ID NO: 259 - protein, 7 aa, synthetic construct
  REGION 1..7: note = Homo sapiensIL330398 VL CDR2 PRT
KDTERPS

SEQ ID NO: 260 - protein, 11 aa, synthetic construct
  REGION 1..11: note = Homo sapiensIL330398 VL CDR3 PRT
LSSDASGASRV

SEQ ID NO: 261 - DNA, 351 bp, synthetic construct; identical to SEQ ID NO: 211
  misc_feature 1..351: note = Homo sapiensIL330398_fgl VH DNA
  source 1..351: mol_type = other DNA

SEQ ID NO: 262 - protein, 117 aa, synthetic construct; identical to SEQ ID NO: 212
  REGION 1..117: note = Homo sapiensIL330398_fgl VH PRT

SEQ ID NO: 263 - protein, 5 aa, synthetic construct
  REGION 1..5: note = Homo sapiensIL330398_fgl VH CDR1 PRT
SYAMS

SEQ ID NO: 264 - protein, 17 aa, synthetic construct
  REGION 1..17: note = Homo sapiensIL330398_fgl VH CDR2 PRT
ASTPWQGSTYYADSVKG

SEQ ID NO: 265 - protein, 8 aa, synthetic construct
  REGION 1..8: note = Homo sapiensIL330398_fgl VH CDR3 PRT
WYWGWIDS

SEQ ID NO: 266 - DNA, 324 bp, synthetic construct
  misc_feature 1..324: note = Homo sapiensIL330398_fgl VL DNA
  source 1..324: mol_type = other DNA
tcctatgagctgatgcagccaccctcggtgtcagtgtccccaggacagacggccaggatcacctgctctggcgatgctttgccaaagcaatatgctcattggtaccagcagaagccaggccaggcccctgtgctggtgatatataaagacactgagaggccctcagggattcctgagcgattctctgggtccagctcagggacaacagtcacgctgaccatcagtggagtccaggcagaagatgaagctgactattactgtttgtccagcgacgcctcgggtgcttcacgggtgttcggcggagggaccaagctgaccgtccta

SEQ ID NO: 267 - protein, 108 aa, synthetic construct
  REGION 1..108: note = Homo sapiensIL330398_fgl VL PRT
SYELMQPPSVSVSPGQTARITCSGDALPKQYAHWYQQKPGQAPVLVIYKDTERPSGIPERFSGSSSGTTVTLTISGVQAEDEADYYCLSSDASGASRVFGGGTKLTVL

SEQ ID NO: 268 - protein, 11 aa, synthetic construct
  REGION 1..11: note = Homo sapiensIL330398_fgl VL CDR1 PRT
SGDALPKQYAH

SEQ ID NO: 269 - protein, 7 aa, synthetic construct
  REGION 1..7: note = Homo sapiensIL330398_fgl VL CDR2 PRT
KDTERPS

SEQ ID NO: 270 - protein, 11 aa, synthetic construct
  REGION 1..11: note = Homo sapiensIL330398_fgl VL CDR3 PRT
LSSDASGASRV

SEQ ID NO: 271 - DNA, 378 bp, synthetic construct
  misc_feature 1..378: note = Homo sapiens33v20064 VH DNA
  source 1..378: mol_type = other DNA
gaggtgcagctgttggagtctgggggaggcttggtacagcctggggggtccctgagactctcctgtgcagcctctggattcacctttagcagctatgccatgagctgggtccgccaggctccagggaaggggctggagtgggtctcagctattagtggtagtggtggtagcacatactacgcagactccgtgaagggccggttcaccatctccagagacaattccaagaacacgctgtatctgcaaatgaacagcctgagagccgaggacacggccgtgtattactgtgcgagagatctgtggatacagctatggggggggggcttgcgttatcccttcggctactggggccaagggacaatggtcaccgtctcgagt

SEQ ID NO: 272 - protein, 126 aa, synthetic construct
  REGION 1..126: note = Homo sapiens33v20064 VH PRT
EVQLLESGGGLVQPGGSLRLSCAASGFTFSSYAMSWVRQAPGKGLEWVSAISGSGGSTYYADSVKGRFTISRDNSKNTLYLQMNSLRAEDTAVYYCARDLWIQLWGGGLRYPFGYWGQGTMVTVSS

SEQ ID NO: 273 - protein, 5 aa, synthetic construct
  REGION 1..5: note = Homo sapiens33v20064 VH CDR1 PRT
SYAMS

SEQ ID NO: 274 - protein, 17 aa, synthetic construct
  REGION 1..17: note = Homo sapiens33v20064 VH CDR2 PRT
AISGSGGSTYYADSVKG

SEQ ID NO: 275 - protein, 17 aa, synthetic construct
  REGION 1..17: note = Homo sapiens33v20064 VH CDR3 PRT
DLWIQLWGGGLRYPFGY

SEQ ID NO: 276 - DNA, 318 bp, synthetic construct
  misc_feature 1..318: note = Homo sapiens33v20064 VL DNA
  source 1..318: mol_type = other DNA
ctgcctgtgctgactcagccaccctcagtgtccgtgtccccaggacagaaggccagcatcacctgctctggagaaagaatgggggataaatatgctgcctggtatcagcagaagccaggccagtcacctatactggtcatctatcaagatacaaagcggccctcagggatccctgagcgattctctggctccaactctgggaacacagccacgttgaccatcagcgggacccaggacatggatgaggctgactattactgtcaggtgtgggacagcagcactggggtattcggcggagggaccaaggtcaccgtccta

SEQ ID NO: 277 - protein, 106 aa, synthetic construct
  REGION 1..106: note = Homo sapiens33v20064 VL PRT
LPVLTQPPSVSVSPGQKASITCSGERMGDKYAAWYQQKPGQSPILVIYQDTKRPSGIPERFSGSNSGNTATLTISGTQDMDEADYYCQVWDSSTGVFGGGTKVTVL

SEQ ID NO: 278 - protein, 11 aa, synthetic construct
  REGION 1..11: note = Homo sapiens33v20064 VL CDR1 PRT
SGERMGDKYAA

SEQ ID NO: 279 - protein, 7 aa, synthetic construct
  REGION 1..7: note = Homo sapiens33v20064 VL CDR2 PRT
QDTKRPS

SEQ ID NO: 280 - protein, 9 aa, synthetic construct
  REGION 1..9: note = Homo sapiens33v20064 VL CDR3 PRT
QVWDSSTGV

SEQ ID NO: 281 - DNA, 378 bp, synthetic construct; identical to SEQ ID NO: 271
  misc_feature 1..378: note = Homo sapiens33_640001 VH DNA
  source 1..378: mol_type = other DNA

SEQ ID NO: 282 - protein, 126 aa, synthetic construct; identical to SEQ ID NO: 272
  REGION 1..126: note = Homo sapiens33_640001 VH PRT

SEQ ID NO: 283 - protein, 5 aa, synthetic construct
  REGION 1..5: note = Homo sapiens33_640001 VH CDR1 PRT
SYAMS

SEQ ID NO: 284 - protein, 17 aa, synthetic construct
  REGION 1..17: note = Homo sapiens33_640001 VH CDR2 PRT
AISGSGGSTYYADSVKG

SEQ ID NO: 285 - protein, 17 aa, synthetic construct
  REGION 1..17: note = Homo sapiens33_640001 VH CDR3 PRT
DLWIQLWGGGLRYPFGY

SEQ ID NO: 286 - DNA, 318 bp, synthetic construct
  misc_feature 1..318: note = Homo sapiens33_640001 VL DNA
  source 1..318: mol_type = other DNA
tcctacgtgctgactcagccaccctcagtgtccgtgtccccaggacagacggccagcatcacctgctctggagaaagaatgggggataaatatgctgcctggtatcagcagaagccaggccagtcacctgtgctggtcatctatcaagatacaaagcggccctcagggatccctgagcgattctctggctccaactctgggaacacagccacgttgaccatcagcgggacccaggccatggatgaggctgactattactgtcaggtgtgggacagcagcactggggtattcggcggagggaccaaggtcaccgtccta

SEQ ID NO: 287 - protein, 106 aa, synthetic construct
  REGION 1..106: note = Homo sapiens33_640001 VL PRT
SYVLTQPPSVSVSPGQTASITCSGERMGDKYAAWYQQKPGQSPVLVIYQDTKRPSGIPERFSGSNSGNTATLTISGTQAMDEADYYCQVWDSSTGVFGGGTKVTVL

SEQ ID NO: 288 - protein, 11 aa, synthetic construct
  REGION 1..11: note = Homo sapiens33_640001 VL CDR1 PRT
SGERMGDKYAA

SEQ ID NO: 289 - protein, 7 aa, synthetic construct
  REGION 1..7: note = Homo sapiens33_640001 VL CDR2 PRT
QDTKRPS

SEQ ID NO: 290 - protein, 9 aa, synthetic construct
  REGION 1..9: note = Homo sapiens33_640001 VL CDR3 PRT
QVWDSSTGV

SEQ ID NO: 291 - DNA, 378 bp, synthetic construct
  misc_feature 1..378: note = Homo sapiens33_640027 VH DNA
  source 1..378: mol_type = other DNA
gaggtgcagctgttggagtctgggggagacttggtacagcctggggggtccctgagactctcctgtgcagcctctggattcacctttagcagctatgccatgagctgggtccgccaggctccagggaaggggctggagtgggtctcagctattggtggtagtggtggtagcacatactacgcagactccgtgaagggccggttcaccatctccagagacaattccaagaacacgctgtatctgcaaatgaacagcctgagagccgaggacacggccgtgtattactgtgcgagagatctgtggatgcagctatggggggggggcttgcgttatcccttcggctactggggccaagggacaatggtcaccgtctcgagt

SEQ ID NO: 292 - protein, 126 aa, synthetic construct
  REGION 1..126: note = Homo sapiens33_640027 VH PRT
EVQLLESGGDLVQPGGSLRLSCAASGFTFSSYAMSWVRQAPGKGLEWVSAIGGSGGSTYYADSVKGRFTISRDNSKNTLYLQMNSLRAEDTAVYYCARDLWMQLWGGGLRYPFGYWGQGTMVTVSS

SEQ ID NO: 293 - protein, 5 aa, synthetic construct
  REGION 1..5: note = Homo sapiens33_640027 VH CDR1 PRT
SYAMS

SEQ ID NO: 294 - protein, 17 aa, synthetic construct
  REGION 1..17: note = Homo sapiens33_640027 VH CDR2 PRT
AIGGSGGSTYYADSVKG

SEQ ID NO: 295 - protein, 17 aa, synthetic construct
  REGION 1..17: note = Homo sapiens33_640027 VH CDR3 PRT
DLWMQLWGGGLRYPFGY

SEQ ID NO: 296 - DNA, 318 bp, synthetic construct
  misc_feature 1..318: note = Homo sapiens33_640027 VL DNA
  source 1..318: mol_type = other DNA
ctgcctgtgctgactcagccaccctcagtgtccgtgtccccaggacagaaggccagcatcacctgctctggagaaagaataggggataaatatgccgcctggtatcagcagaagccgggccagtcacctatactggtcatctatcgagatacaaagcggccctcagggatccctgagcgattctctggctccaactctgggaacacagccacgttgaccatcagcgggacccaggacatggatgaggctgactattactgtcaggtgtgggacagcagcactggggtattcggcggagggaccaaggtcaccgtccta

SEQ ID NO: 297 - protein, 106 aa, synthetic construct
  REGION 1..106: note = Homo sapiens33_640027 VL PRT
LPVLTQPPSVSVSPGQKASITCSGERIGDKYAAWYQQKPGQSPILVIYRDTKRPSGIPERFSGSNSGNTATLTISGTQDMDEADYYCQVWDSSTGVFGGGTKVTVL

SEQ ID NO: 298 - protein, 11 aa, synthetic construct
  REGION 1..11: note = Homo sapiens33_640027 VL CDR1 PRT
SGERIGDKYAA

SEQ ID NO: 299 - protein, 7 aa, synthetic construct
  REGION 1..7: note = Homo sapiens33_640027 VL CDR2 PRT
RDTKRPS

SEQ ID NO: 300 - protein, 9 aa, synthetic construct
  REGION 1..9: note = Homo sapiens33_640027 VL CDR3 PRT
QVWDSSTGV

SEQ ID NO: 301 - DNA, 378 bp, synthetic construct
  misc_feature 1..378: note = Homo sapiens33_640050 VH DNA
  source 1..378: mol_type = other DNA
gaggtgcagctgttggagtctgggggaggcttggtacagcctggggggtccctgagactctcctgtgcagcctctggattcacctttagcagctatgccatgagctgggtccgccaggctccagggaaggggctggagtgggtctcagctattagtggtagtggtggtagcacatactacgcagactccgtgaagggccggttcaccatctccagagacaattccaagaacacgctgtatctgcaaatgaacagcctgagagccgaggacacggccgtgtattactgtccgaggcacaagttcatgcagctatggggggggggcttgcgttatcccttcggctactggggccaagggacaatggtcaccgtctcgagt

SEQ ID NO: 302 - protein, 126 aa, synthetic construct
  REGION 1..126: note = Homo sapiens33_640050 VH PRT
EVQLLESGGGLVQPGGSLRLSCAASGFTFSSYAMSWVRQAPGKGLEWVSAISGSGGSTYYADSVKGRFTISRDNSKNTLYLQMNSLRAEDTAVYYCPRHKFMQLWGGGLRYPFGYWGQGTMVTVSS

SEQ ID NO: 303 - protein, 5 aa, synthetic construct
  REGION 1..5: note = Homo sapiens33_640050 VH CDR1 PRT
SYAMS

SEQ ID NO: 304 - protein, 17 aa, synthetic construct
  REGION 1..17: note = Homo sapiens33_640050 VH CDR2 PRT
AISGSGGSTYYADSVKG

SEQ ID NO: 305 - protein, 17 aa, synthetic construct
  REGION 1..17: note = Homo sapiens33_640050 VH CDR3 PRT
HKFMQLWGGGLRYPFGY

SEQ ID NO: 306 - DNA, 318 bp, synthetic construct; identical to SEQ ID NO: 286
  misc_feature 1..318: note = Homo sapiens33_640050 VL DNA
  source 1..318: mol_type = other DNA

SEQ ID NO: 307 - protein, 106 aa, synthetic construct; identical to SEQ ID NO: 287
  REGION 1..106: note = Homo sapiens33_640050 VL PRT

SEQ ID NO: 308 - protein, 11 aa, synthetic construct
  REGION 1..11: note = Homo sapiens33_640050 VL CDR1 PRT
SGERMGDKYAA

SEQ ID NO: 309 - protein, 7 aa, synthetic construct
  REGION 1..7: note = Homo sapiens33_640050 VL CDR2 PRT
QDTKRPS

SEQ ID NO: 310 - protein, 9 aa, synthetic construct
  REGION 1..9: note = Homo sapiens33_640050 VL CDR3 PRT
QVWDSSTGV

SEQ ID NO: 311 - DNA, 378 bp, synthetic construct
  misc_feature 1..378: note = Homo sapiens33_640047 VH DNA
  source 1..378: mol_type = other DNA
gaggtgcagctgttggagtctgggggaggcttggtacagcctggggggtccctgagactctcctgtgcagcctctggattcacctttagcagctatgccatgagctgggtccgccaggctccagggaaggggctggagtgggtctcagctattagtggtagtggtggtagcacatactacgcagactccgtgaagggccggttcaccatctccagagacaattccaagaacacgctgtatctgcaaatgaacagcctgagagccgaggacacggccgtgtattactgtacgaggctcaagttcatgcagctatggggggggggcttgcgttatcccttcggctactggggccaagggacaatggtcaccgtctcgagt

SEQ ID NO: 312 - protein, 126 aa, synthetic construct
  REGION 1..126: note = Homo sapiens33_640047 VH PRT
EVQLLESGGGLVQPGGSLRLSCAASGFTFSSYAMSWVRQAPGKGLEWVSAISGSGGSTYYADSVKGRFTISRDNSKNTLYLQMNSLRAEDTAVYYCTRLKFMQLWGGGLRYPFGYWGQGTMVTVSS

SEQ ID NO: 313 - protein, 5 aa, synthetic construct
  REGION 1..5: note = Homo sapiens33_640047 VH CDR1 PRT
SYAMS

SEQ ID NO: 314 - protein, 17 aa, synthetic construct
  REGION 1..17: note = Homo sapiens33_640047 VH CDR2 PRT
AISGSGGSTYYADSVKG

SEQ ID NO: 315 - protein, 17 aa, synthetic construct
  REGION 1..17: note = Homo sapiens33_640047 VH CDR3 PRT
LKFMQLWGGGLRYPFGY

SEQ ID NO: 316 - DNA, 318 bp, synthetic construct; identical to SEQ ID NO: 286
  misc_feature 1..318: note = Homo sapiens33_640047 VL DNA
  source 1..318: mol_type = other DNA

SEQ ID NO: 317 - protein, 106 aa, synthetic construct; identical to SEQ ID NO: 287
  REGION 1..106: note = Homo sapiens33_640047 VL PRT

SEQ ID NO: 318 - protein, 11 aa, synthetic construct
  REGION 1..11: note = Homo sapiens33_640047 VL CDR1 PRT
SGERMGDKYAA

SEQ ID NO: 319 - protein, 7 aa, synthetic construct
  REGION 1..7: note = Homo sapiens33_640047 VL CDR2 PRT
QDTKRPS

SEQ ID NO: 320 - protein, 9 aa, synthetic construct
  REGION 1..9: note = Homo sapiens33_640047 VL CDR3 PRT
QVWDSSTGV

SEQ ID NO: 321 - DNA, 384 bp, synthetic construct
  misc_feature 1..384: note = Homo sapiens33_640166 VH DNA
  source 1..384: mol_type = other DNA
gaggtgcagctgttggagtctgggggaggcttggtacagcctggggggtccctgagactctcctgtgcagcctctggattcacctttagcagctatgccatgagctgggtccgccaggctccagggaaggggctggagtgggtctcagctattaatggtgatggtgatggtgggcgcccatactacgcagactccgtgaagggccggttcaccatctccagagacaattccaagaacacgctgtatctgcaaatgaacagcctgagagccgaggacacggccgtgtattactgtgcgagagatctgtggatacagctatggggggggggcttgcgttatcccttcggctactggggccaagggacaatggtcaccgtctcgagt

SEQ ID NO: 322 - protein, 128 aa, synthetic construct
  REGION 1..128: note = Homo sapiens33_640166 VH PRT
EVQLLESGGGLVQPGGSLRLSCAASGFTFSSYAMSWVRQAPGKGLEWVSAINGDGDGGRPYYADSVKGRFTISRDNSKNTLYLQMNSLRAEDTAVYYCARDLWIQLWGGGLRYPFGYWGQGTMVTVSS

SEQ ID NO: 323 - protein, 5 aa, synthetic construct
  REGION 1..5: note = Homo sapiens33_640166 VH CDR1 PRT
SYAMS

SEQ ID NO: 324 - protein, 19 aa, synthetic construct
  REGION 1..19: note = Homo sapiens33_640166 VH CDR2 PRT
AINGDGDGGRPYYADSVKG

SEQ ID NO: 325 - protein, 17 aa, synthetic construct
  REGION 1..17: note = Homo sapiens33_640166 VH CDR3 PRT
DLWIQLWGGGLRYPFGY

SEQ ID NO: 326 - DNA, 318 bp, synthetic construct; identical to SEQ ID NO: 286
  misc_feature 1..318: note = Homo sapiens33_640166 VL DNA
  source 1..318: mol_type = other DNA

SEQ ID NO: 327 - protein, 106 aa, synthetic construct; identical to SEQ ID NO: 287
  REGION 1..106: note = Homo sapiens33_640166 VL PRT

SEQ ID NO: 328 - protein, 11 aa, synthetic construct
  REGION 1..11: note = Homo sapiens33_640166 VL CDR1 PRT
SGERMGDKYAA

SEQ ID NO: 329 - protein, 7 aa, synthetic construct
  REGION 1..7: note = Homo sapiens33_640166 VL CDR2 PRT
QDTKRPS

SEQ ID NO: 330 - protein, 9 aa, synthetic construct
  REGION 1..9: note = Homo sapiens33_640166 VL CDR3 PRT
QVWDSSTGV

SEQ ID NO: 331 - DNA, 378 bp, synthetic construct
  misc_feature 1..378: note = Homo sapiens33_640169 VH DNA
  source 1..378: mol_type = other DNA
gaggtgcagctgttggagtctgggggaggcttggtacagcctggggggtccctgagactctcctgtgcagcctctggattcacctttagcagctatgccatgagctgggtccgccaggctccagggaaggggctggagtgggtctcaggtattagtggtatcgacacaagcacatactacgcagactccgtgaagggccggttcaccatctccagagacaattccaagaacacgctgtatctgcaaatgaacagcctgagagccgaggacacggccgtgtattactgtgcgagagatctgtggatacagctatggggggggggcttgcgttatcccttcggctactggggccaagggacaatggtcaccgtctcgagt

SEQ ID NO: 332 - protein, 126 aa, synthetic construct
  REGION 1..126: note = Homo sapiens33_640169 VH PRT
EVQLLESGGGLVQPGGSLRLSCAASGFTFSSYAMSWVRQAPGKGLEWVSGISGIDTSTYYADSVKGRFTISRDNSKNTLYLQMNSLRAEDTAVYYCARDLWIQLWGGGLRYPFGYWGQGTMVTVSS

SEQ ID NO: 333 - protein, 5 aa, synthetic construct
  REGION 1..5: note = Homo sapiens33_640169 VH CDR1 PRT
SYAMS

SEQ ID NO: 334 - protein, 17 aa, synthetic construct
  REGION 1..17: note = Homo sapiens33_640169 VH CDR2 PRT
GISGIDTSTYYADSVKG

SEQ ID NO: 335 - protein, 17 aa, synthetic construct
  REGION 1..17: note = Homo sapiens33_640169 VH CDR3 PRT
DLWIQLWGGGLRYPFGY

SEQ ID NO: 336 - DNA, 318 bp, synthetic construct; identical to SEQ ID NO: 286
  misc_feature 1..318: note = Homo sapiens33_640169 VL DNA
  source 1..318: mol_type = other DNA

SEQ ID NO: 337 - protein, 106 aa, synthetic construct; identical to SEQ ID NO: 287
  REGION 1..106: note = Homo sapiens33_640169 VL PRT

SEQ ID NO: 338 - protein, 11 aa, synthetic construct
  REGION 1..11: note = Homo sapiens33_640169 VL CDR1 PRT
SGERMGDKYAA

SEQ ID NO: 339 - protein, 7 aa, synthetic construct
  REGION 1..7: note = Homo sapiens33_640169 VL CDR2 PRT
QDTKRPS

SEQ ID NO: 340 - protein, 9 aa, synthetic construct
  REGION 1..9: note = Homo sapiens33_640169 VL CDR3 PRT
QVWDSSTGV

SEQ ID NO: 341 - DNA, 378 bp, synthetic construct
  misc_feature 1..378: note = Homo sapiens33_640170 VH DNA
  source 1..378: mol_type = other DNA
gaggtgcagctgttggagtctgggggaggcttggtacagcctggggggtccctgagactctcctgtgcagcctctggattcacctttagcagctatgccatgagctgggtccgccaggctccagggaaggggctggagtgggtctcaggcatttctgcaatagaccaaagcacatactacgcagactccgtgaagggccggttcaccatctccagagacaattccaagaacacgctgtatctgcaaatgaacagcctgagagccgaggacacggccgtgtattactgtgcgagagatctgtggatacagctatggggggggggcttgcgttatcccttcggctactggggccaagggacaatggtcaccgtctcgagt

SEQ ID NO: 342 - protein, 126 aa, synthetic construct
  REGION 1..126: note = Homo sapiens33_640170 VH PRT
EVQLLESGGGLVQPGGSLRLSCAASGFTFSSYAMSWVRQAPGKGLEWVSGISAIDQSTYYADSVKGRFTISRDNSKNTLYLQMNSLRAEDTAVYYCARDLWIQLWGGGLRYPFGYWGQGTMVTVSS

SEQ ID NO: 343 - protein, 5 aa, synthetic construct
  REGION 1..5: note = Homo sapiens33_640170 VH CDR1 PRT
SYAMS

SEQ ID NO: 344 - protein, 17 aa, synthetic construct
  REGION 1..17: note = Homo sapiens33_640170 VH CDR2 PRT
GISAIDQSTYYADSVKG

SEQ ID NO: 345 - protein, 17 aa, synthetic construct
  REGION 1..17: note = Homo sapiens33_640170 VH CDR3 PRT
DLWIQLWGGGLRYPFGY

SEQ ID NO: 346 - DNA, 318 bp, synthetic construct; identical to SEQ ID NO: 286
  misc_feature 1..318: note = Homo sapiens33_640170 VL DNA
  source 1..318: mol_type = other DNA

SEQ ID NO: 347 - protein, 106 aa, synthetic construct; identical to SEQ ID NO: 287
  REGION 1..106: note = Homo sapiens33_640170 VL PRT

SEQ ID NO: 348 - protein, 11 aa, synthetic construct
  REGION 1..11: note = Homo sapiens33_640170 VL CDR1 PRT
SGERMGDKYAA

SEQ ID NO: 349 - protein, 7 aa, synthetic construct
  REGION 1..7: note = Homo sapiens33_640170 VL CDR2 PRT
QDTKRPS

SEQ ID NO: 350 - protein, 9 aa, synthetic construct
  REGION 1..9: note = Homo sapiens33_640170 VL CDR3 PRT
QVWDSSTGV

SEQ ID NO: 351 - DNA, 378 bp, synthetic construct
  misc_feature 1..378: note = Homo sapiens33_640036 VH DNA
  source 1..378: mol_type = other DNA
gaggtgcagctgttggagtctgggggaggcttggtacagcctggggggtccctgagactctcctgtgcagcctctggattcacctttagcagctatgccatgagctgggtccgccaggctccagggaaggggctggagtgggtctcagctattagtggtagtggtggtagcacatactacgcagactccgtgaagggccggttcaccatctccagagacaattccaagaacacgctgtatctgcaaatgaacagcctgagagccgaggacacggccgtgtattactgtgcgagagatctgtggatgcagctatggggggggggcttgcgttatcccttcggctactggggccaagggacaatggtcaccgtctcgagt

SEQ ID NO: 352 - protein, 126 aa, synthetic construct
  REGION 1..126: note = Homo sapiens33_640036 VH PRT
EVQLLESGGGLVQPGGSLRLSCAASGFTFSSYAMSWVRQAPGKGLEWVSAISGSGGSTYYADSVKGRFTISRDNSKNTLYLQMNSLRAEDTAVYYCARDLWMQLWGGGLRYPFGYWGQGTMVTVSS

SEQ ID NO: 353 - protein, 5 aa, synthetic construct
  REGION 1..5: note = Homo sapiens33_640036 VH CDR1 PRT
SYAMS

SEQ ID NO: 354 - protein, 17 aa, synthetic construct
  REGION 1..17: note = Homo sapiens33_640036 VH CDR2 PRT
AISGSGGSTYYADSVKG

SEQ ID NO: 355 - protein, 17 aa, synthetic construct
  REGION 1..17: note = Homo sapiens33_640036 VH CDR3 PRT
DLWMQLWGGGLRYPFGY

SEQ ID NO: 356 - DNA, 318 bp, synthetic construct
  misc_feature 1..318: note = Homo sapiens33_640036 VL DNA
  source 1..318: mol_type = other DNA
tcctacgtgctgactcagccaccctcagtgtccgtgtccccaggacagacggccagcatcacctgctctggagaaagaatgggggataaatatgctgcctggtatcagcagaagccaggccagtcacctgtgctggtcatctatcgagatacaaagcggccctcagggatccctgagcgattctctggctccaactctgggaacacagccacgttgaccatcagcgggacccaggccatggatgaggctgactattactgtcaggtgtgggacagcagcactggggtattcggcggagggaccaaggtcaccgtccta

SEQ ID NO: 357 - protein, 106 aa, synthetic construct
  REGION 1..106: note = Homo sapiens33_640036 VL PRT
SYVLTQPPSVSVSPGQTASITCSGERMGDKYAAWYQQKPGQSPVLVIYRDTKRPSGIPERFSGSNSGNTATLTISGTQAMDEADYYCQVWDSSTGVFGGGTKVTVL

SEQ ID NO: 358 - protein, 11 aa, synthetic construct
  REGION 1..11: note = Homo sapiens33_640036 VL CDR1 PRT
SGERMGDKYAA

SEQ ID NO: 359 - protein, 7 aa, synthetic construct
  REGION 1..7: note = Homo sapiens33_640036 VL CDR2 PRT
RDTKRPS

SEQ ID NO: 360 - protein, 9 aa, synthetic construct
  REGION 1..9: note = Homo sapiens33_640036 VL CDR3 PRT
QVWDSSTGV

SEQ ID NO: 361 - DNA, 378 bp, synthetic construct; identical to SEQ ID NO: 311
  misc_feature 1..378: note = Homo sapiens33_640117 VH DNA
  source 1..378: mol_type = other DNA

SEQ ID NO: 362 - protein, 126 aa, synthetic construct; identical to SEQ ID NO: 312
  REGION 1..126: note = Homo sapiens33_640117 VH PRT

SEQ ID NO: 363 - protein, 5 aa, synthetic construct
  REGION 1..5: note = Homo sapiens33_640117 VH CDR1 PRT
SYAMS

SEQ ID NO: 364 - protein, 17 aa, synthetic construct
  REGION 1..17: note = Homo sapiens33_640117 VH CDR2 PRT
AISGSGGSTYYADSVKG

SEQ ID NO: 365 - protein, 17 aa, synthetic construct
  REGION 1..17: note = Homo sapiens33_640117 VH CDR3 PRT
LKFMQLWGGGLRYPFGY

SEQ ID NO: 366 - DNA, 318 bp, synthetic construct; identical to SEQ ID NO: 356
  misc_feature 1..318: note = Homo sapiens33_640117 VL DNA
  source 1..318: mol_type = other DNA

SEQ ID NO: 367 - protein, 106 aa, synthetic construct; identical to SEQ ID NO: 357
  REGION 1..106: note = Homo sapiens33_640117 VL PRT

SEQ ID NO: 368 - protein, 11 aa, synthetic construct
  REGION 1..11: note = Homo sapiens33_640117 VL CDR1 PRT
SGERMGDKYAA

SEQ ID NO: 369 - protein, 7 aa, synthetic construct
  REGION 1..7: note = Homo sapiens33_640117 VL CDR2 PRT
RDTKRPS

SEQ ID NO: 370 - protein, 9 aa, synthetic construct
  REGION 1..9: note = Homo sapiens33_640117 VL CDR3 PRT
QVWDSSTGV

SEQ ID NO: 371 - DNA, 378 bp, synthetic construct
  misc_feature 1..378: note = Homo sapiens33_640076 VH DNA
  source 1..378: mol_type = other DNA
gaggtgcagctgttggagtctgggggaggcttggtacagcctggggggtccctgagactctcctgtgcagcctctggattcacctttagcagctatgccatgagctgggtccgccgggctccagggaaggggctggagtgggtctcagctattagtggtagtggtggtagcacatactacgcagactccgtgaagggccggttcaccatctccagagacaattccaagaacacgctgtatctgcaaatgaacagcctgagagccgaggacacggccgtgtattactgtgcgagagatctgtggatggagaactgggtggggggcttgcgttatcccttcggctactggggccaagggacaatggtcaccgtctcgagt

SEQ ID NO: 372 - protein, 126 aa, synthetic construct
  REGION 1..126: note = Homo sapiens33_640076 VH PRT
EVQLLESGGGLVQPGGSLRLSCAASGFTFSSYAMSWVRRAPGKGLEWVSAISGSGGSTYYADSVKGRFTISRDNSKNTLYLQMNSLRAEDTAVYYCARDLWMENWVGGLRYPFGYWGQGTMVTVSS

SEQ ID NO: 373 - protein, 5 aa, synthetic construct
  REGION 1..5: note = Homo sapiens33_640076 VH CDR1 PRT
SYAMS

SEQ ID NO: 374 - protein, 17 aa, synthetic construct
  REGION 1..17: note = Homo sapiens33_640076 VH CDR2 PRT
AISGSGGSTYYADSVKG

SEQ ID NO: 375 - protein, 17 aa, synthetic construct
  REGION 1..17: note = Homo sapiens33_640076 VH CDR3 PRT
DLWMENWVGGLRYPFGY

SEQ ID NO: 376 - DNA, 318 bp, synthetic construct
  misc_feature 1..318: note = Homo sapiens33_640076 VL DNA
  source 1..318: mol_type = other DNA
tcctacgtgctgactcagccaccctcagtgtccgtgtcaccaggacagacggccagcatcacctgctctggagaaagaatgggggataaatatgctgcctggtatcagcagaagccaggccagtcacctgtgctggtcatctatcaagatacaaagcggccctcagggatccctgagcgattctctggctccaactctgggaacacagccacgttgaccatcagcgggacccaggccatagatgaggccgactattactgtgaggtcaagaagtccgacactggggtattcggcggagggaccaaggtcaccgtccta

SEQ ID NO: 377 - protein, 106 aa, synthetic construct
  REGION 1..106: note = Homo sapiens33_640076 VL PRT
SYVLTQPPSVSVSPGQTASITCSGERMGDKYAAWYQQKPGQSPVLVIYQDTKRPSGIPERFSGSNSGNTATLTISGTQAIDEADYYCEVKKSDTGVFGGGTKVTVL

SEQ ID NO: 378 - protein, 11 aa, synthetic construct
  REGION 1..11: note = Homo sapiens33_640076 VL CDR1 PRT
SGERMGDKYAA

SEQ ID NO: 379 - protein, 7 aa, synthetic construct
  REGION 1..7: note = Homo sapiens33_640076 VL CDR2 PRT
QDTKRPS

SEQ ID NO: 380 - protein, 9 aa, synthetic construct
  REGION 1..9: note = Homo sapiens33_640076 VL CDR3 PRT
EVKKSDTGV

SEQ ID NO: 381 - DNA, 378 bp, synthetic construct
  misc_feature 1..378: note = Homo sapiens33_640081 VH DNA
  source 1..378: mol_type = other DNA
gaggtgcagctgttggagtctgggggaggctcggtacagcctggggggtccctgagactctcctgtgcagcctctggattcacctttagcagctatgccatgaactgggtccgccaggctccagggaaggggctggagtgggtctcagctattagtggtagtggtggtagcacacactacgcagactccgtgaagggccggttcaccatctccagagacaattccaagaacacgctgtatctgcaaatgaacagcctgagagccgaggacacggccgtgtattactgtggccgggccaagttcatgcagctatggggggggggcttgcgttatcccctcggctactggggccaagggacaatggtcaccgtctcgagt

SEQ ID NO: 382 - protein, 126 aa, synthetic construct
  REGION 1..126: note = Homo sapiens33_640081 VH PRT
EVQLLESGGGSVQPGGSLRLSCAASGFTFSSYAMNWVRQAPGKGLEWVSAISGSGGSTHYADSVKGRFTISRDNSKNTLYLQMNSLRAEDTAVYYCGRAKFMQLWGGGLRYPLGYWGQGTMVTVSS

SEQ ID NO: 383 - protein, 5 aa, synthetic construct
  REGION 1..5: note = Homo sapiens33_640081 VH CDR1 PRT
SYAMN

SEQ ID NO: 384 - protein, 17 aa, synthetic construct
  REGION 1..17: note = Homo sapiens33_640081 VH CDR2 PRT
AISGSGGSTHYADSVKG

SEQ ID NO: 385 - protein, 17 aa, synthetic construct
  REGION 1..17: note = Homo sapiens33_640081 VH CDR3 PRT
AKFMQLWGGGLRYPLGY

SEQ ID NO: 386 - DNA, 321 bp, synthetic construct
  misc_feature 1..321: note = Homo sapiens33_640081 VL DNA
  source 1..321: mol_type = other DNA
tcctacgtgctgactcagccaccctcagtgtccgtgtccccaggacagacggccagcatcacctgctctggagaaagaatgggggataaatatgctgcctggtatcagcagaagccaggccagtcacctgtgctggtcatctatcaagatacaaagcggccctcagggatccctgagcgattctctggctccaactctgggaacacagccacgttgaccatcagcgggacccaggccacggatgaggctgactattactgtcaggtgtgggcggccgacgacactggggtattcggcggagggaccaaggtcaccgtccta

SEQ ID NO: 387 - protein, 107 aa, synthetic construct
  REGION 1..107: note = Homo sapiens33_640081 VL PRT
SYVLTQPPSVSVSPGQTASITCSGERMGDKYAAWYQQKPGQSPVLVIYQDTKRPSGIPERFSGSNSGNTATLTISGTQATDEADYYCQVWAADDTGVFGGGTKVTVL

SEQ ID NO: 388 - protein, 11 aa, synthetic construct
  REGION 1..11: note = Homo sapiens33_640081 VL CDR1 PRT
SGERMGDKYAA

SEQ ID NO: 389 - protein, 7 aa, synthetic construct
  REGION 1..7: note = Homo sapiens33_640081 VL CDR2 PRT
QDTKRPS

SEQ ID NO: 390 - protein, 10 aa, synthetic construct
  REGION 1..10: note = Homo sapiens33_640081 VL CDR3 PRT
QVWAADDTGV

SEQ ID NO: 391 - DNA, 378 bp, synthetic construct
  misc_feature 1..378: note = Homo sapiens33_640082 VH DNA
  source 1..378: mol_type = other DNA
gaggtgcagctgttggagtctgggggaggcttggtacagcctggggggtccctgagactctcctgtgcagcctctggattcacctttagcagctatgccatgagctgggtccgccaggctccagggaaggggctggagtgggtctcagctattagtggtagtggtggtagcacatactacgcagactccgtgaagggccggttcaccatctccagagacaattccaagaacacgctgtatctgcaaatgaacagcctgagagccgaggacacggccgtgtattactgtgcccggcagaagttcatgcagctatggggggggggcttgcgttatcccttcggctactggggccaagggacaatggtcaccgtctcgagt

SEQ ID NO: 392 - protein, 126 aa, synthetic construct
  REGION 1..126: note = Homo sapiens33_640082 VH PRT
EVQLLESGGGLVQPGGSLRLSCAASGFTFSSYAMSWVRQAPGKGLEWVSAISGSGGSTYYADSVKGRFTISRDNSKNTLYLQMNSLRAEDTAVYYCARQKFMQLWGGGLRYPFGYWGQGTMVTVSS

SEQ ID NO: 393 - protein, 5 aa, synthetic construct
  REGION 1..5: note = Homo sapiens33_640082 VH CDR1 PRT
SYAMS

SEQ ID NO: 394 - protein, 17 aa, synthetic construct
  REGION 1..17: note = Homo sapiens33_640082 VH CDR2 PRT
AISGSGGSTYYADSVKG

SEQ ID NO: 395 - protein, 17 aa, synthetic construct
  REGION 1..17: note = Homo sapiens33_640082 VH CDR3 PRT
QKFMQLWGGGLRYPFGY

SEQ ID NO: 396 - DNA, 318 bp, synthetic construct
  misc_feature 1..318: note = Homo sapiens33_640082 VL DNA
  source 1..318: mol_type = other DNA
tcctacgtgctgactcagccaccctcagtgtccgtgtccccagggcagacggccagcatcacctgctctggagaaagaatgggggataaatatgctgcctggtatcagcagaagccaggccagtcacctgtgctggtcatctatcaagatacaaagcggccctcagggatccctgagcgattctctggctccaactctgggaacacagccacgttgaccatcagcgggacccaggccattgatgaggctgactattactgtggcgtgttgaagcaggacactggggtattcggcggagggaccaaggtcaccgtccta

SEQ ID NO: 397 - protein, 106 aa, synthetic construct
  REGION 1..106: note = Homo sapiens33_640082 VL PRT
SYVLTQPPSVSVSPGQTASITCSGERMGDKYAAWYQQKPGQSPVLVIYQDTKRPSGIPERFSGSNSGNTATLTISGTQAIDEADYYCGVLKQDTGVFGGGTKVTVL

SEQ ID NO: 398 - protein, 11 aa, synthetic construct
  REGION 1..11: note = Homo sapiens33_640082 VL CDR1 PRT
SGERMGDKYAA

SEQ ID NO: 399 - protein, 7 aa, synthetic construct
  REGION 1..7: note = Homo sapiens33_640082 VL CDR2 PRT
QDTKRPS

SEQ ID NO: 400 - protein, 9 aa, synthetic construct
  REGION 1..9: note = Homo sapiens33_640082 VL CDR3 PRT
GVLKQDTGV

SEQ ID NO: 401 - DNA, 378 bp, synthetic construct
  misc_feature 1..378: note = Homo sapiens33_640084 VH DNA
  source 1..378: mol_type = other DNA
gaggtgcagctgttggagtctgggggaggcttggtacagcctggggggtccctgagactctcctgtgcggcctctggattcgcctttagcagctatgccatgagctgggtccgccaggctccagggaaggggctggagtgggtctcagctattagtggtagtggtggtagcacatactacgcagactccgtgaagggccggttcaccatctccagagacaattccaagaacacgctgtatctgcaaatgaacagcctgagagccgaggacacggccgtgtattactgtgcccggcagaagttcatgcagctatggggggggggcttgcgttatccctttggctactggggccaagggacaatggtcaccgtctcgagt

SEQ ID NO: 402 - protein, 126 aa, synthetic construct
  REGION 1..126: note = Homo sapiens33_640084 VH PRT
EVQLLESGGGLVQPGGSLRLSCAASGFAFSSYAMSWVRQAPGKGLEWVSAISGSGGSTYYADSVKGRFTISRDNSKNTLYLQMNSLRAEDTAVYYCARQKFMQLWGGGLRYPFGYWGQGTMVTVSS

SEQ ID NO: 403 - protein, 5 aa, synthetic construct
  REGION 1..5: note = Homo sapiens33_640084 VH CDR1 PRT
SYAMS

SEQ ID NO: 404 - protein, 17 aa, synthetic construct
  REGION 1..17: note = Homo sapiens33_640084 VH CDR2 PRT
AISGSGGSTYYADSVKG

SEQ ID NO: 405 - protein, 17 aa, synthetic construct
  REGION 1..17: note = Homo sapiens33_640084 VH CDR3 PRT
QKFMQLWGGGLRYPFGY

SEQ ID NO: 406 - DNA, 318 bp, synthetic construct
  misc_feature 1..318: note = Homo sapiens33_640084 VL DNA
  source 1..318: mol_type = other DNA
tcctacgtgctgactcagccaccctcagtgtccgtgtccccaggacagacggccagcatcacctgctctggagaaagaatgggggataaatatgctgcctggtatcagcagaagccaggccagtcacctgtgctggtcatctatcaagatacaaagcggccctcagggatccctgagcgattctctggctccaactctgggaacacagccacgttgaccatcagcgggacccaggccgtggatgaggctgactattactgtcaggtgtggcgggacgacagccccatcttcggcggagggaccaaggtcaccgtccta

SEQ ID NO: 407 - protein, 106 aa, synthetic construct
  REGION 1..106: note = Homo sapiens33_640084 VL PRT
SYVLTQPPSVSVSPGQTASITCSGERMGDKYAAWYQQKPGQSPVLVIYQDTKRPSGIPERFSGSNSGNTATLTISGTQAVDEADYYCQVWRDDSPIFGGGTKVTVL

SEQ ID NO: 408 - protein, 11 aa, synthetic construct
  REGION 1..11: note = Homo sapiens33_640084 VL CDR1 PRT
SGERMGDKYAA

SEQ ID NO: 409 - protein, 7 aa, synthetic construct
  REGION 1..7: note = Homo sapiens33_640084 VL CDR2 PRT
QDTKRPS

SEQ ID NO: 410 - protein, 9 aa, synthetic construct
  REGION 1..9: note = Homo sapiens33_640084 VL CDR3 PRT
QVWRDDSPI

SEQ ID NO: 411 - DNA, 378 bp, synthetic construct
  misc_feature 1..378: note = Homo sapiens33_640086 VH DNA
  source 1..378: mol_type = other DNA
gaggtgcagctgttggagtctgggggaggcttggtacagcctggtgggtccctgagactctcctgtgcagcctctggattcacctttagcagctatgccatgagctgggtccgccaggctccagggaaggggctggagtgggtctcagctattagtggtagtggtggtagcacatactacgcagactccgtgaagggccggttcaccatcaccagagacaattccaagaacacgctgtatctgcaaatgaacagcctgagagccgaggacacggccgtgtattactgtgcccgcgacaagttcatgcagctatggggggggggcttgcgttatcccttcggctactggggccaagggacaatggtcaccgtctcgagt

SEQ ID NO: 412 - protein, 126 aa, synthetic construct
  REGION 1..126: note = Homo sapiens33_640086 VH PRT
EVQLLESGGGLVQPGGSLRLSCAASGFTFSSYAMSWVRQAPGKGLEWVSAISGSGGSTYYADSVKGRFTITRDNSKNTLYLQMNSLRAEDTAVYYCARDKFMQLWGGGLRYPFGYWGQGTMVTVSS

SEQ ID NO: 413 - protein, 5 aa, synthetic construct
  REGION 1..5: note = Homo sapiens33_640086 VH CDR1 PRT
SYAMS

SEQ ID NO: 414 - protein, 17 aa, synthetic construct
  REGION 1..17: note = Homo sapiens33_640086 VH CDR2 PRT
AISGSGGSTYYADSVKG

SEQ ID NO: 415 - protein, 17 aa, synthetic construct
  REGION 1..17: note = Homo sapiens33_640086 VH CDR3 PRT
DKFMQLWGGGLRYPFGY

SEQ ID NO: 416 - DNA, 318 bp, synthetic construct
  misc_feature 1..318: note = Homo sapiens33_640086 VL DNA
  source 1..318: mol_type = other DNA
tcctacgtgctgactcagccaccctcagtgtccgtgtccccaggacagacggccagcatcacctgctctggagaaagaatgggggataaatatgctgcctggtatcagcagaagccaggccagtcacctgtgctggtcatctatcaagatacaaagcggccctcagggatccctgagcgattctctggctccaactctgggaacacagccacgttgaccatcagcgggacccaagccatggatgaggctgactattactgtgaggtcaaggtgaaggacactggggtattcggcggagggaccaaggtcaccgtccta

SEQ ID NO: 417 - protein, 106 aa, synthetic construct
  REGION 1..106: note = Homo sapiens33_640086 VL PRT
SYVLTQPPSVSVSPGQTASITCSGERMGDKYAAWYQQKPGQSPVLVIYQDTKRPSGIPERFSGSNSGNTATLTISGTQAMDEADYYCEVKVKDTGVFGGGTKVTVL

SEQ ID NO: 418 - protein, 11 aa, synthetic construct
  REGION 1..11: note = Homo sapiens33_640086 VL CDR1 PRT
SGERMGDKYAA

SEQ ID NO: 419 - protein, 7 aa, synthetic construct
  REGION 1..7: note = Homo sapiens33_640086 VL CDR2 PRT
QDTKRPS

SEQ ID NO: 420 - protein, 9 aa, synthetic construct
  REGION 1..9: note = Homo sapiens33_640086 VL CDR3 PRT
EVKVKDTGV

SEQ ID NO: 421 - DNA, 378 bp, synthetic construct
  misc_feature 1..378: note = Homo sapiens33_640087 VH DNA
  source 1..378: mol_type = other DNA
gaggtgcagctgttggagtctgggggaggcttggtacagcctggggggtccctgagactctcctgtgcagcctctggattcacctttagcagctatgccatgagctgggtccgccaggctccagggaaggggctggagtgggtctcagctattagtggtagtggtgatagcacatactacgcagactccgtgaagggccggttcaccatctccagagacaattccaagaacacgctgtatctgcaaatgaacagcctgagagccgaggacacggccgtgtattactgtgcccggcagaagttcatgcagctatggggggggggcttgcgttatcccttcggctactggggccaggggacaatggtcaccgtttcgagt

SEQ ID NO: 422 - protein, 126 aa, synthetic construct
  REGION 1..126: note = Homo sapiens33_640087 VH PRT
EVQLLESGGGLVQPGGSLRLSCAASGFTFSSYAMSWVRQAPGKGLEWVSAISGSGDSTYYADSVKGRFTISRDNSKNTLYLQMNSLRAEDTAVYYCARQKFMQLWGGGLRYPFGYWGQGTMVTVSS

SEQ ID NO: 423 - protein, 5 aa, synthetic construct
  REGION 1..5: note = Homo sapiens33_640087 VH CDR1 PRT
SYAMS

SEQ ID NO: 424 - protein, 17 aa, synthetic construct
  REGION 1..17: note = Homo sapiens33_640087 VH CDR2 PRT
AISGSGDSTYYADSVKG

SEQ ID NO: 425 - protein, 17 aa, synthetic construct
  REGION 1..17: note = Homo sapiens33_640087 VH CDR3 PRT
QKFMQLWGGGLRYPFGY

SEQ ID NO: 426 - DNA, 318 bp, synthetic construct
  misc_feature 1..318: note = Homo sapiens33_640087 VL DNA
  source 1..318: mol_type = other DNA
tcctacgtgctgactcagccaccctcagtgtccgtgtccccaggacaggcggccagcatcacctgctctggagaaggaatgggggataaatatgctgcctggtatcagcagaagccaggccagtcacctgtgctggtcatctatcaagatacaaagcggccctcagggatccctgagcgattctctggctccaactctgggaacacagccacgttgaccatcagcgggacccaggctatggatgaggctgactattactgtggggtgatccaggacaacactggggtattcggcggagggaccaaggtcaccgtccta

SEQ ID NO: 427 - protein, 106 aa, synthetic construct
  REGION 1..106: note = Homo sapiens33_640087 VL PRT
SYVLTQPPSVSVSPGQAASITCSGEGMGDKYAAWYQQKPGQSPVLVIYQDTKRPSGIPERFSGSNSGNTATLTISGTQAMDEADYYCGVIQDNTGVFGGGTKVTVL

SEQ ID NO: 428 - protein, 11 aa, synthetic construct
  REGION 1..11: note = Homo sapiens33_640087 VL CDR1 PRT
SGEGMGDKYAA

SEQ ID NO: 429 - protein, 7 aa, synthetic construct
  REGION 1..7: note = Homo sapiens33_640087 VL CDR2 PRT
QDTKRPS

SEQ ID NO: 430 - protein, 9 aa, synthetic construct
  REGION 1..9: note = Homo sapiens33_640087 VL CDR3 PRT
GVIQDNTGV

SEQ ID NO: 431 - DNA, 378 bp, synthetic construct
  misc_feature 1..378: note = Homo sapiens33_640076-1 VH DNA
  source 1..378: mol_type = other DNA
gaggtgcagctgttggagtctgggggaggcttggtacagcctggggggtccctgagactctcctgtgcagcctctggattcacctttagcagctatgccatgagctgggtccgccaggctccagggaaggggctggagtgggtctcagctattagtggtagtggtggtagcacatactacgcagactccgtgaagggccggttcaccatctccagagacaattccaagaacacgctgtatctgcaaatgaacagcctgagagccgaggacacggccgtgtattactgtgcgagagatctgtggatggagaactgggtggggggcttgcgttatcccttcggctactggggccaagggacaatggtcaccgtctcctca

SEQ ID NO: 432 - protein, 126 aa, synthetic construct
  REGION 1..126: note = Homo sapiens33_640076-1 VH PRT
EVQLLESGGGLVQPGGSLRLSCAASGFTFSSYAMSWVRQAPGKGLEWVSAISGSGGSTYYADSVKGRFTISRDNSKNTLYLQMNSLRAEDTAVYYCARDLWMENWVGGLRYPFGYWGQGTMVTVSS

SEQ ID NO: 433 - protein, 5 aa, synthetic construct
  REGION 1..5: note = Homo sapiens33_640076-1 VH CDR1 PRT
SYAMS

SEQ ID NO: 434 - protein, 17 aa, synthetic construct
  REGION 1..17: note = Homo sapiens33_640076-1 VH CDR2 PRT
AISGSGGSTYYADSVKG

SEQ ID NO: 435 - protein, 17 aa, synthetic construct
  REGION 1..17: note = Homo sapiens33_640076-1 VH CDR3 PRT
DLWMENWVGGLRYPFGY

SEQ ID NO: 436 - DNA, 318 bp, synthetic construct
  misc_feature 1..318: note = Homo sapiens33_640076-1 VL DNA
  source 1..318: mol_type = other DNA
tcctatgtgctgactcagccaccctcagtgtccgtgtcaccaggacagacggccagcatcacctgctctggagaaagaatgggggataaatatgctgcctggtatcagcagaagccaggccagtcacctgtgctggtcatctatcgagatacaaagcggccctcagggatccctgagcgattctctggctccaactctgggaacacagccacgttgaccatcagcgggacccaggccatggatgaggccgactattactgtgaggtcaagaagtccgacactggggtattcggcggagggaccaaggtcaccgtccta

SEQ ID NO: 437 - protein, 106 aa, synthetic construct
  REGION 1..106: note = Homo sapiens33_640076-1 VL PRT
SYVLTQPPSVSVSPGQTASITCSGERMGDKYAAWYQQKPGQSPVLVIYRDTKRPSGIPERFSGSNSGNTATLTISGTQAMDEADYYCEVKKSDTGVFGGGTKVTVL

SEQ ID NO: 438 - protein, 11 aa, synthetic construct
  REGION 1..11: note = Homo sapiens33_640076-1 VL CDR1 PRT
SGERMGDKYAA

SEQ ID NO: 439 - protein, 7 aa, synthetic construct
  REGION 1..7: note = Homo sapiens33_640076-1 VL CDR2 PRT
RDTKRPS

SEQ ID NO: 440 - protein, 9 aa, synthetic construct
  REGION 1..9: note = Homo sapiens33_640076-1 VL CDR3 PRT
EVKKSDTGV

SEQ ID NO: 441 - DNA, 378 bp, synthetic construct
  misc_feature 1..378: note = Homo sapiens33_640081-A VH DNA
  source 1..378: mol_type = other DNA
gaggtgcagctgttggagtctgggggaggcttggtacagcctggggggtccctgagactctcctgtgcagcctctggattcacctttagcagctatgccatgaactgggtccgccaggctccagggaaggggctggagtgggtctcagctattagtggtagtggtggtagcacacactacgcagactccgtgaagggccggttcaccatctccagagacaattccaagaacacgctgtatctgcaaatgaacagcctgagagccgaggacacggccgtgtattactgtggccgggccaagttcatgcagctatggggggggggcttgcgttatcccctcggctactggggccaagggacaatggtcaccgtctcctca

SEQ ID NO: 442 - protein, 126 aa, synthetic construct
  REGION 1..126: note = Homo sapiens33_640081-A VH PRT
EVQLLESGGGLVQPGGSLRLSCAASGFTFSSYAMNWVRQAPGKGLEWVSAISGSGGSTHYADSVKGRFTISRDNSKNTLYLQMNSLRAEDTAVYYCGRAKFMQLWGGGLRYPLGYWGQGTMVTVSS

SEQ ID NO: 443 - protein, 5 aa, synthetic construct
  REGION 1..5: note = Homo sapiens33_640081-A VH CDR1 PRT
SYAMN

SEQ ID NO: 444 - protein, 17 aa, synthetic construct
  REGION 1..17: note = Homo sapiens33_640081-A VH CDR2 PRT
AISGSGGSTHYADSVKG

SEQ ID NO: 445 - protein, 17 aa, synthetic construct
  REGION 1..17: note = Homo sapiens33_640081-A VH CDR3 PRT
AKFMQLWGGGLRYPLGY

SEQ ID NO: 446 - DNA, 321 bp, synthetic construct
  misc_feature 1..321: note = Homo sapiens33_640081-A VL DNA
  source 1..321: mol_type = other DNA
tcctatgtgctgactcagccaccctcagtgtccgtgtccccaggacagacggccagcatcacctgctctggagaaagaatgggggataaatatgctgcctggtatcagcagaagccaggccagtcacctgtgctggtcatctatcgagatacaaagcggccctcagggatccctgagcgattctctggctccaactctgggaacacagccacgttgaccatcagcgggacccaggccatggatgaggctgactattactgtcaggtgtgggcggccgacgacactggggtattcggcggagggaccaaggtcaccgtccta

SEQ ID NO: 447 - protein, 107 aa, synthetic construct
  REGION 1..107: note = Homo sapiens33_640081-A VL PRT
SYVLTQPPSVSVSPGQTASITCSGERMGDKYAAWYQQKPGQSPVLVIYRDTKRPSGIPERFSGSNSGNTATLTISGTQAMDEADYYCQVWAADDTGVFGGGTKVTVL

SEQ ID NO: 448 - protein, 11 aa, synthetic construct
  REGION 1..11: note = Homo sapiens33_640081-A VL CDR1 PRT
SGERMGDKYAA

SEQ ID NO: 449 - protein, 7 aa, synthetic construct
  REGION 1..7: note = Homo sapiens33_640081-A VL CDR2 PRT
RDTKRPS

SEQ ID NO: 450 - protein, 10 aa, synthetic construct
  REGION 1..10: note = Homo sapiens33_640081-A VL CDR3 PRT
QVWAADDTGV

SEQ ID NO: 451 - DNA, 378 bp, synthetic construct; identical to SEQ ID NO: 391
  misc_feature 1..378: note = Homo sapiens33_640082-2 VH DNA
  source 1..378: mol_type = other DNA

SEQ ID NO: 452 - protein, 126 aa, synthetic construct; identical to SEQ ID NO: 392
  REGION 1..126: note = Homo sapiens33_640082-2 VH PRT

SEQ ID NO: 453 - protein, 5 aa, synthetic construct
  REGION 1..5: note = Homo sapiens33_640082-2 VH CDR1 PRT
SYAMS

SEQ ID NO: 454 - protein, 17 aa, synthetic construct
  REGION 1..17: note = Homo sapiens33_640082-2 VH CDR2 PRT
AISGSGGSTYYADSVKG

SEQ ID NO: 455 - protein, 17 aa, synthetic construct
  REGION 1..17: note = Homo sapiens33_640082-2 VH CDR3 PRT
QKFMQLWGGGLRYPFGY

SEQ ID NO: 456 - DNA, 318 bp, synthetic construct
  misc_feature 1..318: note = Homo sapiens33_640082-2 VL DNA
  source 1..318: mol_type = other DNA
tcctatgtgctgactcagccaccctcagtgtccgtgtccccagggcagacggccagcatcacctgctctggagaaagaatgggggataaatatgctgcctggtatcagcagaagccaggccagtcacctgtgctggtcatctatcgagatacaaagcggccctcagggatccctgagcgattctctggctccaactctgggaacacagccacgttgaccatcagcgggacccaggccatggatgaggctgactattactgtggcgtgttgaagcaggacactggggtattcggcggagggaccaaggtcaccgtccta

SEQ ID NO: 457 - protein, 106 aa, synthetic construct
  REGION 1..106: note = Homo sapiens33_640082-2 VL PRT
SYVLTQPPSVSVSPGQTASITCSGERMGDKYAAWYQQKPGQSPVLVIYRDTKRPSGIPERFSGSNSGNTATLTISGTQAMDEADYYCGVLKQDTGVFGGGTKVTVL

SEQ ID NO: 458 - protein, 11 aa, synthetic construct
  REGION 1..11: note = Homo sapiens33_640082-2 VL CDR1 PRT
SGERMGDKYAA

SEQ ID NO: 459 - protein, 7 aa, synthetic construct
  REGION 1..7: note = Homo sapiens33_640082-2 VL CDR2 PRT
RDTKRPS

SEQ ID NO: 460 - protein, 9 aa, synthetic construct
  REGION 1..9: note = Homo sapiens33_640082-2 VL CDR3 PRT
GVLKQDTGV

SEQ ID NO: 461 - DNA, 378 bp, synthetic construct; identical to SEQ ID NO: 401
  misc_feature 1..378: note = Homo sapiens33_640084-2 VH DNA
  source 1..378: mol_type = other DNA

SEQ ID NO: 462 - protein, 126 aa, synthetic construct; identical to SEQ ID NO: 402
  REGION 1..126: note = Homo sapiens33_640084-2 VH PRT

SEQ ID NO: 463 - protein, 5 aa, synthetic construct
  REGION 1..5: note = Homo sapiens33_640084-2 VH CDR1 PRT
SYAMS

SEQ ID NO: 464 - protein, 17 aa, synthetic construct
  REGION 1..17: note = Homo sapiens33_640084-2 VH CDR2 PRT
AISGSGGSTYYADSVKG

SEQ ID NO: 465 - protein, 17 aa, synthetic construct
  REGION 1..17: note = Homo sapiens33_640084-2 VH CDR3 PRT
QKFMQLWGGGLRYPFGY

SEQ ID NO: 466 - DNA, 318 bp, synthetic construct
  misc_feature 1..318: note = Homo sapiens33_640084-2 VL DNA
  source 1..318: mol_type = other DNA
tcctatgtgctgactcagccaccctcagtgtccgtgtccccaggacagacggccagcatcacctgctctggagaaagaatgggggataaatatgctgcctggtatcagcagaagccaggccagtcacctgtgctggtcatctatcgagatacaaagcggccctcagggatccctgagcgattctctggctccaactctgggaacacagccacgttgaccatcagcgggacccaggccatggatgaggctgactattactgtcaggtgtggcgggacgacagccccatcttcggcggagggaccaaggtcaccgtccta

SEQ ID NO: 467 - protein, 106 aa, synthetic construct
  REGION 1..106: note = Homo sapiens33_640084-2 VL PRT
SYVLTQPPSVSVSPGQTASITCSGERMGDKYAAWYQQKPGQSPVLVIYRDTKRPSGIPERFSGSNSGNTATLTISGTQAMDEADYYCQVWRDDSPIFGGGTKVTVL

SEQ ID NO: 468 - protein, 11 aa, synthetic construct
  REGION 1..11: note = Homo sapiens33_640084-2 VL CDR1 PRT
SGERMGDKYAA

SEQ ID NO: 469 - protein, 7 aa, synthetic construct
  REGION 1..7: note = Homo sapiens33_640084-2 VL CDR2 PRT
RDTKRPS

SEQ ID NO: 470 - protein, 9 aa, synthetic construct
  REGION 1..9: note = Homo sapiens33_640084-2 VL CDR3 PRT
QVWRDDSPI

SEQ ID NO: 471 - DNA, 378 bp, synthetic construct
  misc_feature 1..378: note = Homo sapiens33_640086-2 VH DNA
  source 1..378: mol_type = other DNA
gaggtgcagctgttggagtctgggggaggcttggtacagcctggtgggtccctgagactctcctgtgcagcctctggattcacctttagcagctatgccatgagctgggtccgccaggctccagggaaggggctggagtgggtctcagctattagtggtagtggtggtagcacatactacgcagactccgtgaagggccggttcaccatcagcagagacaattccaagaacacgctgtatctgcaaatgaacagcctgagagccgaggacacggccgtgtattactgtgcccgcgacaagttcatgcagctatggggggggggcttgcgttatcccttcggctactggggccaagggacaatggtcaccgtctcctca

SEQ ID NO: 472 - protein, 126 aa, synthetic construct
  REGION 1..126: note = Homo sapiens33_640086-2 VH PRT
EVQLLESGGGLVQPGGSLRLSCAASGFTFSSYAMSWVRQAPGKGLEWVSAISGSGGSTYYADSVKGRFTISRDNSKNTLYLQMNSLRAEDTAVYYCARDKFMQLWGGGLRYPFGYWGQGTMVTVSS

SEQ ID NO: 473 - protein, 5 aa, synthetic construct
  REGION 1..5: note = Homo sapiens33_640086-2 VH CDR1 PRT
SYAMS

SEQ ID NO: 474 - protein, 17 aa, synthetic construct
  REGION 1..17: note = Homo sapiens33_640086-2 VH CDR2 PRT
AISGSGGSTYYADSVKG

SEQ ID NO: 475 - protein, 17 aa, synthetic construct
  REGION 1..17: note = Homo sapiens33_640086-2 VH CDR3 PRT
DKFMQLWGGGLRYPFGY

SEQ ID NO: 476 - DNA, 318 bp, synthetic construct
  misc_feature 1..318: note = Homo sapiens33_640086-2 VL DNA
  source 1..318: mol_type = other DNA
tcctatgtgctgactcagccaccctcagtgtccgtgtccccaggacagacggccagcatcacctgctctggagaaagaatgggggataaatatgctgcctggtatcagcagaagccaggccagtcacctgtgctggtcatctatcgagatacaaagcggccctcagggatccctgagcgattctctggctccaactctgggaacacagccacgttgaccatcagcgggacccaagccatggatgaggctgactattactgtgaggtcaaggtgaaggacactggggtattcggcggagggaccaaggtcaccgtccta

SEQ ID NO: 477 - protein, 106 aa, synthetic construct
  REGION 1..106: note = Homo sapiens33_640086-2 VL PRT
SYVLTQPPSVSVSPGQTASITCSGERMGDKYAAWYQQKPGQSPVLVIYRDTKRPSGIPERFSGSNSGNTATLTISGTQAMDEADYYCEVKVKDTGVFGGGTKVTVL

SEQ ID NO: 478 - protein, 11 aa, synthetic construct
  REGION 1..11: note = Homo sapiens33_640086-2 VL CDR1 PRT
SGERMGDKYAA

SEQ ID NO: 479 - protein, 7 aa, synthetic construct
  REGION 1..7: note = Homo sapiens33_640086-2 VL CDR2 PRT
RDTKRPS

SEQ ID NO: 480 - protein, 9 aa, synthetic construct
  REGION 1..9: note = Homo sapiens33_640086-2 VL CDR3 PRT
EVKVKDTGV

SEQ ID NO: 481 - DNA, 378 bp, synthetic construct; identical to SEQ ID NO: 421
  misc_feature 1..378: note = Homo sapiens33_640087-2 VH DNA
  source 1..378: mol_type = other DNA

SEQ ID NO: 482 - protein, 126 aa, synthetic construct; identical to SEQ ID NO: 422
  REGION 1..126: note = Homo sapiens33_640087-2 VH PRT

SEQ ID NO: 483 - protein, 5 aa, synthetic construct
  REGION 1..5: note = Homo sapiens33_640087-2 VH CDR1 PRT
SYAMS

SEQ ID NO: 484 - protein, 17 aa, synthetic construct
  REGION 1..17: note = Homo sapiens33_640087-2 VH CDR2 PRT
AISGSGDSTYYADSVKG

SEQ ID NO: 485 - protein, 17 aa, synthetic construct
  REGION 1..17: note = Homo sapiens33_640087-2 VH CDR3 PRT
QKFMQLWGGGLRYPFGY

SEQ ID NO: 486 - DNA, 318 bp, synthetic construct
  misc_feature 1..318: note = Homo sapiens33_640087-2 VL DNA
  source 1..318: mol_type = other DNA
tcctatgtgctgactcagccaccctcagtgtccgtgtccccaggacagacggccagcatcacctgctctggagaaggaatgggggataaatatgctgcctggtatcagcagaagccaggccagtcacctgtgctggtcatctatcgagatacaaagcggccctcagggatccctgagcgattctctggctccaactctgggaacacagccacgttgaccatcagcgggacccaggctatggatgaggctgactattactgtggggtgatccaggacaacactggggtattcggcggagggaccaaggtcaccgtccta

SEQ ID NO: 487 - protein, 106 aa, synthetic construct
  REGION 1..106: note = Homo sapiens33_640087-2 VL PRT
SYVLTQPPSVSVSPGQTASITCSGEGMGDKYAAWYQQKPGQSPVLVIYRDTKRPSGIPERFSGSNSGNTATLTISGTQAMDEADYYCGVIQDNTGVFGGGTKVTVL

SEQ ID NO: 488 - protein, 11 aa, synthetic construct
  REGION 1..11: note = Homo sapiens33_640087-2 VL CDR1 PRT
SGEGMGDKYAA

SEQ ID NO: 489 - protein, 7 aa, synthetic construct
  REGION 1..7: note = Homo sapiens33_640087-2 VL CDR2 PRT
RDTKRPS

SEQ ID NO: 490 - protein, 9 aa, synthetic construct
  REGION 1..9: note = Homo sapiens33_640087-2 VL CDR3 PRT
GVIQDNTGV

SEQ ID NO: 491 - DNA, 378 bp, synthetic construct
  misc_feature 1..378: note = Homo sapiens33_640076-4 VH DNA
  source 1..378: mol_type = other DNA
gaggtgcagctgttggagtctgggggaggcttggtacagcctggggggtccctgagactctcctgtgcagcctctggattcacctttagcagctatgccatgagctgggtccgccaggctccagggaaggggctggagtgggtctcaggcatttctgcaatagaccaaagcacatactacgcagactccgtgaagggccggttcaccatctccagagacaattccaagaacacgctgtatctgcaaatgaacagcctgagagccgaggacacggccgtgtattactgtgcgagagatctgtggatggagaactgggtggggggcttgcgttatcccttcggctactggggccaagggacaatggtcaccgtctcctca

SEQ ID NO: 492 - protein, 126 aa, synthetic construct
  REGION 1..126: note = Homo sapiens33_640076-4 VH PRT
EVQLLESGGGLVQPGGSLRLSCAASGFTFSSYAMSWVRQAPGKGLEWVSGISAIDQSTYYADSVKGRFTISRDNSKNTLYLQMNSLRAEDTAVYYCARDLWMENWVGGLRYPFGYWGQGTMVTVSS

SEQ ID NO: 493 - protein, 5 aa, synthetic construct
  REGION 1..5: note = Homo sapiens33_640076-4 VH CDR1 PRT
SYAMS

SEQ ID NO: 494 - protein, 17 aa, synthetic construct
  REGION 1..17: note = Homo sapiens33_640076-4 VH CDR2 PRT
GISAIDQSTYYADSVKG

SEQ ID NO: 495 - protein, 17 aa, synthetic construct
  REGION 1..17: note = Homo sapiens33_640076-4 VH CDR3 PRT
DLWMENWVGGLRYPFGY

SEQ ID NO: 496 - DNA, 318 bp, synthetic construct; identical to SEQ ID NO: 436
  misc_feature 1..318: note = Homo sapiens33_640076-4 VL DNA
  source 1..318: mol_type = other DNA

SEQ ID NO: 497 - protein, 106 aa, synthetic construct; identical to SEQ ID NO: 437
  REGION 1..106: note = Homo sapiens33_640076-4 VL PRT

SEQ ID NO: 498 - protein, 11 aa, synthetic construct
  REGION 1..11: note = Homo sapiens33_640076-4 VL CDR1 PRT
SGERMGDKYAA

SEQ ID NO: 499 - protein, 7 aa, synthetic construct
  REGION 1..7: note = Homo sapiens33_640076-4 VL CDR2 PRT
RDTKRPS

SEQ ID NO: 500 - protein, 9 aa, synthetic construct
  REGION 1..9: note = Homo sapiens33_640076-4 VL CDR3 PRT
EVKKSDTGV

SEQ ID NO: 501 - DNA, 384 bp, synthetic construct
  misc_feature 1..384: note = Homo sapiens33_640082-4 VH DNA
  source 1..384: mol_type = other DNA
gaggtgcagctgttggagtctgggggaggcttggtacagcctggggggtccctgagactctcctgtgcagcctctggattcacctttagcagctatgccatgagctgggtccgccaggctccagggaaggggctggagtgggtctcagctattaatggtgatggtgatggtgggcgcccatactacgcagactccgtgaagggccggttcaccatctccagagacaattccaagaacacgctgtatctgcaaatgaacagcctgagagccgaggacacggccgtgtattactgtgcccggcagaagttcatgcagctatggggggggggcttgcgttatcccttcggctactggggccaagggacaatggtcaccgtctcctca

SEQ ID NO: 502 - protein, 128 aa, synthetic construct
  REGION 1..128: note = Homo sapiens33_640082-4 VH PRT
EVQLLESGGGLVQPGGSLRLSCAASGFTFSSYAMSWVRQAPGKGLEWVSAINGDGDGGRPYYADSVKGRFTISRDNSKNTLYLQMNSLRAEDTAVYYCARQKFMQLWGGGLRYPFGYWGQGTMVTVSS

SEQ ID NO: 503 - protein, 5 aa, synthetic construct
  REGION 1..5: note = Homo sapiens33_640082-4 VH CDR1 PRT
SYAMS

SEQ ID NO: 504 - protein, 19 aa, synthetic construct
  REGION 1..19: note = Homo sapiens33_640082-4 VH CDR2 PRT
AINGDGDGGRPYYADSVKG

SEQ ID NO: 505 - protein, 17 aa, synthetic construct
  REGION 1..17: note = Homo sapiens33_640082-4 VH CDR3 PRT
QKFMQLWGGGLRYPFGY

SEQ ID NO: 506 - DNA, 318 bp, synthetic construct; identical to SEQ ID NO: 456
  misc_feature 1..318: note = Homo sapiens33_640082-4 VL DNA
  source 1..318: mol_type = other DNA

SEQ ID NO: 507 - protein, 106 aa, synthetic construct; identical to SEQ ID NO: 457
  REGION 1..106: note = Homo sapiens33_640082-4 VL PRT

SEQ ID NO: 508 - protein, 11 aa, synthetic construct
  REGION 1..11: note = Homo sapiens33_640082-4 VL CDR1 PRT
SGERMGDKYAA

SEQ ID NO: 509 - protein, 7 aa, synthetic construct
  REGION 1..7: note = Homo sapiens33_640082-4 VL CDR2 PRT
RDTKRPS

SEQ ID NO: 510 - protein, 9 aa, synthetic construct
  REGION 1..9: note = Homo sapiens33_640082-4 VL CDR3 PRT
GVLKQDTGV

SEQ ID NO: 511 - DNA, 378 bp, synthetic construct
  misc_feature 1..378: note = Homo sapiens33_640082-6 VH DNA
  source 1..378: mol_type = other DNA
gaggtgcagctgttggagtctgggggaggcttggtacagcctggggggtccctgagactctcctgtgcagcctctggattcacctttagcagctatgccatgagctgggtccgccaggctccagggaaggggctggagtgggtctcaggtattagtggtatcgacacaagcacatactacgcagactccgtgaagggccggttcaccatctccagagacaattccaagaacacgctgtatctgcaaatgaacagcctgagagccgaggacacggccgtgtattactgtgcccggcagaagttcatgcagctatggggggggggcttgcgttatcccttcggctactggggccaagggacaatggtcaccgtctcctca

SEQ ID NO: 512 - protein, 126 aa, synthetic construct
  REGION 1..126: note = Homo sapiens33_640082-6 VH PRT
EVQLLESGGGLVQPGGSLRLSCAASGFTFSSYAMSWVRQAPGKGLEWVSGISGIDTSTYYADSVKGRFTISRDNSKNTLYLQMNSLRAEDTAVYYCARQKFMQLWGGGLRYPFGYWGQGTMVTVSS

SEQ ID NO: 513 - protein, 5 aa, synthetic construct
  REGION 1..5: note = Homo sapiens33_640082-6 VH CDR1 PRT
SYAMS

SEQ ID NO: 514 - protein, 17 aa, synthetic construct
  REGION 1..17: note = Homo sapiens33_640082-6 VH CDR2 PRT
GISGIDTSTYYADSVKG

SEQ ID NO: 515 - protein, 17 aa, synthetic construct
  REGION 1..17: note = Homo sapiens33_640082-6 VH CDR3 PRT
QKFMQLWGGGLRYPFGY

SEQ ID NO: 516 - DNA, 318 bp, synthetic construct; identical to SEQ ID NO: 456
  misc_feature 1..318: note = Homo sapiens33_640082-6 VL DNA
  source 1..318: mol_type = other DNA

SEQ ID NO: 517 - protein, 106 aa, synthetic construct; identical to SEQ ID NO: 457
  REGION 1..106: note = Homo sapiens33_640082-6 VL PRT

SEQ ID NO: 518 - protein, 11 aa, synthetic construct
  REGION 1..11: note = Homo sapiens33_640082-6 VL CDR1 PRT
SGERMGDKYAA

SEQ ID NO: 519 - protein, 7 aa, synthetic construct
  REGION 1..7: note = Homo sapiens33_640082-6 VL CDR2 PRT
RDTKRPS

SEQ ID NO: 520 - protein, 9 aa, synthetic construct
  REGION 1..9: note = Homo sapiens33_640082-6 VL CDR3 PRT
GVLKQDTGV

SEQ ID NO: 521 - DNA, 378 bp, synthetic construct
  misc_feature 1..378: note = Homo sapiens33_640082-7 VH DNA
  source 1..378: mol_type = other DNA
gaggtgcagctgttggagtctgggggaggcttggtacagcctggggggtccctgagactctcctgtgcagcctctggattcacctttagcagctatgccatgagctgggtccgccaggctccagggaaggggctggagtgggtctcaggcatttctgcaatagaccaaagcacatactacgcagactccgtgaagggccggttcaccatctccagagacaattccaagaacacgctgtatctgcaaatgaacagcctgagagccgaggacacggccgtgtattactgtgcccggcagaagttcatgcagctatggggggggggcttgcgttatcccttcggctactggggccaagggacaatggtcaccgtctcctca

SEQ ID NO: 522 - protein, 126 aa, synthetic construct
  REGION 1..126: note = Homo sapiens33_640082-7 VH PRT
EVQLLESGGGLVQPGGSLRLSCAASGFTFSSYAMSWVRQAPGKGLEWVSGISAIDQSTYYADSVKGRFTISRDNSKNTLYLQMNSLRAEDTAVYYCARQKFMQLWGGGLRYPFGYWGQGTMVTVSS

SEQ ID NO: 523 - protein, 5 aa, synthetic construct
  REGION 1..5: note = Homo sapiens33_640082-7 VH CDR1 PRT
SYAMS

SEQ ID NO: 524 - protein, 17 aa, synthetic construct
  REGION 1..17: note = Homo sapiens33_640082-7 VH CDR2 PRT
GISAIDQSTYYADSVKG

SEQ ID NO: 525 - protein, 17 aa, synthetic construct
  REGION 1..17: note = Homo sapiens33_640082-7 VH CDR3 PRT
QKFMQLWGGGLRYPFGY

SEQ ID NO: 526 - DNA, 318 bp, synthetic construct; identical to SEQ ID NO: 456
  misc_feature 1..318: note = Homo sapiens33_640082-7 VL DNA
  source 1..318: mol_type = other DNA

SEQ ID NO: 527 - protein, 106 aa, synthetic construct; identical to SEQ ID NO: 457
  REGION 1..106: note = Homo sapiens33_640082-7 VL PRT

SEQ ID NO: 528 - protein, 11 aa, synthetic construct
  REGION 1..11: note = Homo sapiens33_640082-7 VL CDR1 PRT
SGERMGDKYAA

SEQ ID NO: 529 - protein, 7 aa, synthetic construct
  REGION 1..7: note = Homo sapiens33_640082-7 VL CDR2 PRT
RDTKRPS

SEQ ID NO: 530 - protein, 9 aa, synthetic construct
  REGION 1..9: note = Homo sapiens33_640082-7 VL CDR3 PRT
GVLKQDTGV

SEQ ID NO: 531 - DNA, 378 bp, synthetic construct
  misc_feature 1..378: note = Homo sapiens33_640086-6 VH DNA
  source 1..378: mol_type = other DNA
gaggtgcagctgttggagtctgggggaggcttggtacagcctggtgggtccctgagactctcctgtgcagcctctggattcacctttagcagctatgccatgagctgggtccgccaggctccagggaaggggctggagtgggtctcaggtattagtggtatcgacacaagcacatactacgcagactccgtgaagggccggttcaccatcagcagagacaattccaagaacacgctgtatctgcaaatgaacagcctgagagccgaggacacggccgtgtattactgtgcccgcgacaagttcatgcagctatggggggggggcttgcgttatcccttcggctactggggccaagggacaatggtcaccgtctcctca

SEQ ID NO: 532 - protein, 126 aa, synthetic construct
  REGION 1..126: note = Homo sapiens33_640086-6 VH PRT
EVQLLESGGGLVQPGGSLRLSCAASGFTFSSYAMSWVRQAPGKGLEWVSGISGIDTSTYYADSVKGRFTISRDNSKNTLYLQMNSLRAEDTAVYYCARDKFMQLWGGGLRYPFGYWGQGTMVTVSS

SEQ ID NO: 533 - protein, 5 aa, synthetic construct
  REGION 1..5: note = Homo sapiens33_640086-6 VH CDR1 PRT
SYAMS

SEQ ID NO: 534 - protein, 17 aa, synthetic construct
  REGION 1..17: note = Homo sapiens33_640086-6 VH CDR2 PRT
GISGIDTSTYYADSVKG

SEQ ID NO: 535 - protein, 17 aa, synthetic construct
  REGION 1..17: note = Homo sapiens33_640086-6 VH CDR3 PRT
DKFMQLWGGGLRYPFGY

SEQ ID NO: 536 - DNA, 318 bp, synthetic construct; identical to SEQ ID NO: 476
  misc_feature 1..318: note = Homo sapiens33_640086-6 VL DNA
  source 1..318: mol_type = other DNA

SEQ ID NO: 537 - protein, 106 aa, synthetic construct; identical to SEQ ID NO: 477
  REGION 1..106: note = Homo sapiens33_640086-6 VL PRT

SEQ ID NO: 538 - protein, 11 aa, synthetic construct
  REGION 1..11: note = Homo sapiens33_640086-6 VL CDR1 PRT
SGERMGDKYAA

SEQ ID NO: 539 - protein, 7 aa, synthetic construct
  REGION 1..7: note = Homo sapiens33_640086-6 VL CDR2 PRT
RDTKRPS

SEQ ID NO: 540 - protein, 9 aa, synthetic construct
  REGION 1..9: note = Homo sapiens33_640086-6 VL CDR3 PRT
EVKVKDTGV

SEQ ID NO: 541 - DNA, 378 bp, synthetic construct
  misc_feature 1..378: note = Homo sapiens33_640087-7 VH DNA
  source 1..378: mol_type = other DNA
gaggtgcagctgttggagtctgggggaggcttggtacagcctggggggtccctgagactctcctgtgcagcctctggattcacctttagcagctatgccatgagctgggtccgccaggctccagggaaggggctggagtgggtctcaggcatttctgcaatagaccaaagcacatactacgcagactccgtgaagggccggttcaccatctccagagacaattccaagaacacgctgtatctgcaaatgaacagcctgagagccgaggacacggccgtgtattactgtgcccggcagaagttcatgcagctatggggggggggcttgcgttatcccttcggctactggggccaggggacaatggtcaccgtctcctca

SEQ ID NO: 542 - protein, 126 aa, synthetic construct; identical to SEQ ID NO: 522
  REGION 1..126: note = Homo sapiens33_640087-7 VH PRT

SEQ ID NO: 543 - protein, 5 aa, synthetic construct
  REGION 1..5: note = Homo sapiens33_640087-7 VH CDR1 PRT
SYAMS

SEQ ID NO: 544 - protein, 17 aa, synthetic construct
  REGION 1..17: note = Homo sapiens33_640087-7 VH CDR2 PRT
GISAIDQSTYYADSVKG

SEQ ID NO: 545 - protein, 17 aa, synthetic construct
  REGION 1..17: note = Homo sapiens33_640087-7 VH CDR3 PRT
QKFMQLWGGGLRYPFGY

SEQ ID NO: 546 - DNA, 318 bp, synthetic construct; identical to SEQ ID NO: 486
  misc_feature 1..318: note = Homo sapiens33_640087-7 VL DNA
  source 1..318: mol_type = other DNA

SEQ ID NO: 547 - protein, 106 aa, synthetic construct; identical to SEQ ID NO: 487
  REGION 1..106: note = Homo sapiens33_640087-7 VL PRT

SEQ ID NO: 548 - protein, 11 aa, synthetic construct
  REGION 1..11: note = Homo sapiens33_640087-7 VL CDR1 PRT
SGEGMGDKYAA

SEQ ID NO: 549 - protein, 7 aa, synthetic construct
  REGION 1..7: note = Homo sapiens33_640087-7 VL CDR2 PRT
RDTKRPS

SEQ ID NO: 550 - protein, 9 aa, synthetic construct
  REGION 1..9: note = Homo sapiens33_640087-7 VL CDR3 PRT
GVIQDNTGV

SEQ ID NO: 551 - DNA, 378 bp, synthetic construct
  misc_feature 1..378: note = Homo sapiens33_640201 VH DNA
  source 1..378: mol_type = other DNA
gaggtgcagctgttggagtctgggggaggcttggtacagcctggggggtccctgagactctcctgtgcagcctctggattcacctttagcagctatgccatgagctgggtccgccaggctccagggaaggggctggagtgggtctcatcaattgacgccattagttcaagcacatactacgcagactccgtgaagggccggttcaccatctccagagacaattccaagaacacgctgtatctgcaaatgaacagcctgagagccgaggacacggccgtgtattactgttcccgccagaagttcatgcagctatggggggggggcttgcgttatcccttcggctactggggccaagggacaatggtcaccgtctcgagt

SEQ ID NO: 552 - protein, 126 aa, synthetic construct
  REGION 1..126: note = Homo sapiens33_640201 VH PRT
EVQLLESGGGLVQPGGSLRLSCAASGFTFSSYAMSWVRQAPGKGLEWVSSIDAISSSTYYADSVKGRFTISRDNSKNTLYLQMNSLRAEDTAVYYCSRQKFMQLWGGGLRYPFGYWGQGTMVTVSS

SEQ ID NO: 553 - protein, 5 aa, synthetic construct
  REGION 1..5: note = Homo sapiens33_640201 VH CDR1 PRT
SYAMS

SEQ ID NO: 554 - protein, 17 aa, synthetic construct
  REGION 1..17: note = Homo sapiens33_640201 VH CDR2 PRT
SIDAISSSTYYADSVKG

SEQ ID NO: 555 - protein, 17 aa, synthetic construct
  REGION 1..17: note = Homo sapiens33_640201 VH CDR3 PRT
QKFMQLWGGGLRYPFGY

SEQ ID NO: 556 - DNA, 318 bp, synthetic construct
  misc_feature 1..318: note = Homo sapiens33_640201 VL DNA
  source 1..318: mol_type = other DNA
tcctacgtgctgactcagccaccctcagtgtccgtgtccccaggacagacggccagcatcacctgctctggagaaagaatgggggataaatatgctgcctggtatcagcagaagccaggccagtcacctgtgctggtcatctatcaagatacaaagcggccctcagggatccctgagcgattctctggctccaactctgggaacacagccacgttgaccatcagcgggacccaggccgtggatgaggctgactattactgtggcgtgttgaagcaggacactggggtattcggcggagggaccaaggtcaccgtccta

SEQ ID NO: 557 - protein, 106 aa, synthetic construct
  REGION 1..106: note = Homo sapiens33_640201 VL PRT
SYVLTQPPSVSVSPGQTASITCSGERMGDKYAAWYQQKPGQSPVLVIYQDTKRPSGIPERFSGSNSGNTATLTISGTQAVDEADYYCGVLKQDTGVFGGGTKVTVL

SEQ ID NO: 558 - protein, 11 aa, synthetic construct
  REGION 1..11: note = Homo sapiens33_640201 VL CDR1 PRT
SGERMGDKYAA

SEQ ID NO: 559 - protein, 7 aa, synthetic construct
  REGION 1..7: note = Homo sapiens33_640201 VL CDR2 PRT
QDTKRPS

SEQ ID NO: 560 - protein, 9 aa, synthetic construct
  REGION 1..9: note = Homo sapiens33_640201 VL CDR3 PRT
GVLKQDTGV

SEQ ID NO: 561 - DNA, 378 bp, synthetic construct
  misc_feature 1..378: note = Homo sapiens33_640237 VH DNA
  source 1..378: mol_type = other DNA
gaggtgcagctgttggaatctgggggaggcttggtacagcctggggggtccctgagactctcctgtgcagcctctggattcacctttagcagctatgccatgagctgggtccgccaggctccagggaaggggctggagtgggtctcaggcattgcagacgatttcaccagcacatactacgcagaccccgtgaagggccggttcaccatctccagagacaattccaagaacacgctgtatctgcaaatgaacagcctgagagccgaggacacggccgtgtattactgtgcgagagatctgtggatgatgaactacgcgggcggcttgcgttatcccttcggctactggggccaagggacaacggtcaccgtctcgagt

SEQ ID NO: 562 - protein, 126 aa, synthetic construct
  REGION 1..126: note = Homo sapiens33_640237 VH PRT
EVQLLESGGGLVQPGGSLRLSCAASGFTFSSYAMSWVRQAPGKGLEWVSGIADDFTSTYYADPVKGRFTISRDNSKNTLYLQMNSLRAEDTAVYYCARDLWMMNYAGGLRYPFGYWGQGTTVTVSS

SEQ ID NO: 563 - protein, 5 aa, synthetic construct
  REGION 1..5: note = Homo sapiens33_640237 VH CDR1 PRT
SYAMS

SEQ ID NO: 564 - protein, 17 aa, synthetic construct
  REGION 1..17: note = Homo sapiens33_640237 VH CDR2 PRT
GIADDFTSTYYADPVKG

SEQ ID NO: 565 - protein, 17 aa, synthetic construct
  REGION 1..17: note = Homo sapiens33_640237 VH CDR3 PRT
DLWMMNYAGGLRYPFGY

SEQ ID NO: 566 - DNA, 318 bp, synthetic construct
  misc_feature 1..318: note = Homo sapiens33_640237 VL DNA
  source 1..318: mol_type = other DNA
tcctacgtgctgactcagccaccctcagtgtccgtgtccccaggacagacggccagcatcacctgctctggagaaagaatgggggataaatatgctgcctggtatcagcagaagccaggccagtcacctgtgctggtcatctatcgagatacaaagcggccctcagggatccctgagcgattctctggctccaactctgggaacacagccacgttgaccatcagcgggacccaggccattgatgaggctgactattactgtggcgtgttgaagcaggacactggggtattcggcggagggaccaaggtcaccgtccta

SEQ ID NO: 567 - protein, 106 aa, synthetic construct
  REGION 1..106: note = Homo sapiens33_640237 VL PRT
SYVLTQPPSVSVSPGQTASITCSGERMGDKYAAWYQQKPGQSPVLVIYRDTKRPSGIPERFSGSNSGNTATLTISGTQAIDEADYYCGVLKQDTGVFGGGTKVTVL

SEQ ID NO: 568 - protein, 11 aa, synthetic construct
  REGION 1..11: note = Homo sapiens33_640237 VL CDR1 PRT
SGERMGDKYAA

SEQ ID NO: 569 - protein, 7 aa, synthetic construct
  REGION 1..7: note = Homo sapiens33_640237 VL CDR2 PRT
RDTKRPS

SEQ ID NO: 570 - protein, 9 aa, synthetic construct
  REGION 1..9: note = Homo sapiens33_640237 VL CDR3 PRT
GVLKQDTGV

SEQ ID NO: 571 - DNA, 378 bp, synthetic construct; identical to SEQ ID NO: 551
  misc_feature 1..378: note = Homo sapiens33_640201-2 VH DNA
  source 1..378: mol_type = other DNA

SEQ ID NO: 572 - protein, 126 aa, synthetic construct; identical to SEQ ID NO: 552
  REGION 1..126: note = Homo sapiens33_640201-2 VH PRT

SEQ ID NO: 573 - protein, 5 aa, synthetic construct
  REGION 1..5: note = Homo sapiens33_640201-2 VH CDR1 PRT
SYAMS

SEQ ID NO: 574 - protein, 17 aa, synthetic construct
  REGION 1..17: note = Homo sapiens33_640201-2 VH CDR2 PRT
SIDAISSSTYYADSVKG

SEQ ID NO: 575 - protein, 17 aa, synthetic construct
  REGION 1..17: note = Homo sapiens33_640201-2 VH CDR3 PRT
QKFMQLWGGGLRYPFGY

SEQ ID NO: 576 - DNA, 318 bp, synthetic construct
  misc_feature 1..318: note = Homo sapiens33_640201-2 VL DNA
  source 1..318: mol_type = other DNA
tcctatgtgctgactcagccaccctcagtgtccgtgtccccaggacagacggccagcatcacctgctctggagaaagaatgggggataaatatgctgcctggtatcagcagaagccaggccagtcacctgtgctggtcatctatcgagatacaaagcggccctcagggatccctgagcgattctctggctccaactctgggaacacagccacgttgaccatcagcgggacccaggccatggatgaggctgactattactgtggcgtgttgaagcaggacactggggtattcggcggagggaccaaggtcaccgtccta

SEQ ID NO: 577 - protein, 106 aa, synthetic construct; identical to SEQ ID NO: 457
  REGION 1..106: note = Homo sapiens33_640201-2 VL PRT

SEQ ID NO: 578 - protein, 11 aa, synthetic construct
  REGION 1..11: note = Homo sapiens33_640201-2 VL CDR1 PRT
SGERMGDKYAA

SEQ ID NO: 579 - protein, 7 aa, synthetic construct
  REGION 1..7: note = Homo sapiens33_640201-2 VL CDR2 PRT
RDTKRPS

SEQ ID NO: 580 - protein, 9 aa, synthetic construct
  REGION 1..9: note = Homo sapiens33_640201-2 VL CDR3 PRT
GVLKQDTGV

SEQ ID NO: 581 - DNA, 378 bp, synthetic construct
  misc_feature 1..378: note = Homo sapiens33_640237-2 VH DNA
  source 1..378: mol_type = other DNA
gaggtgcagctgttggagtctgggggaggcttggtacagcctggggggtccctgagactctcctgtgcagcctctggattcacctttagcagctatgccatgagctgggtccgccaggctccagggaaggggctggagtgggtctcaggcattgcagacgatttcaccagcacatactacgcagaccccgtgaagggccggttcaccatctccagagacaattccaagaacacgctgtatctgcaaatgaacagcctgagagccgaggacacggccgtgtattactgtgcgagagatctgtggatgatgaactacgcgggcggcttgcgttatcccttcggctactggggccaagggaccatggtcaccgtctcctca

SEQ ID NO: 582 - protein, 126 aa, synthetic construct
  REGION 1..126: note = Homo sapiens33_640237-2 VH PRT
EVQLLESGGGLVQPGGSLRLSCAASGFTFSSYAMSWVRQAPGKGLEWVSGIADDFTSTYYADPVKGRFTISRDNSKNTLYLQMNSLRAEDTAVYYCARDLWMMNYAGGLRYPFGYWGQGTMVTVSS

SEQ ID NO: 583 - protein, 5 aa, synthetic construct
  REGION 1..5: note = Homo sapiens33_640237-2 VH CDR1 PRT
SYAMS

SEQ ID NO: 584 - protein, 17 aa, synthetic construct
  REGION 1..17: note = Homo sapiens33_640237-2 VH CDR2 PRT
GIADDFTSTYYADPVKG

SEQ ID NO: 585 - protein, 17 aa, synthetic construct
  REGION 1..17: note = Homo sapiens33_640237-2 VH CDR3 PRT
DLWMMNYAGGLRYPFGY

SEQ ID NO: 586 - DNA, 318 bp, synthetic construct; identical to SEQ ID NO: 576
  misc_feature 1..318: note = Homo sapiens33_640237-2 VL DNA
  source 1..318: mol_type = other DNA

SEQ ID NO: 587 - protein, 106 aa, synthetic construct; identical to SEQ ID NO: 457
  REGION 1..106: note = Homo sapiens33_640237-2 VL PRT

SEQ ID NO: 588 - protein, 11 aa, synthetic construct
  REGION 1..11: note = Homo sapiens33_640237-2 VL CDR1 PRT
SGERMGDKYAA

SEQ ID NO: 589 - protein, 7 aa, synthetic construct
  REGION 1..7: note = Homo sapiens33_640237-2 VL CDR2 PRT
RDTKRPS

SEQ ID NO: 590 - protein, 9 aa, synthetic construct
  REGION 1..9: note = Homo sapiens33_640237-2 VL CDR3 PRT
GVLKQDTGV

SEQ ID NO: 591 - DNA, 378 bp, synthetic construct; identical to SEQ ID NO: 491
  misc_feature 1..378: note = Homo sapiens33_640076-4B VH DNA
  source 1..378: mol_type = other DNA

SEQ ID NO: 592 - protein, 126 aa, synthetic construct; identical to SEQ ID NO: 492
  REGION 1..126: note = Homo sapiens33_640076-4B VH PRT

SEQ ID NO: 593 - DNA, 318 bp, synthetic construct
  misc_feature 1..318: note = Homo sapiens33_640076-4B VL DNA
  source 1..318: mol_type = other DNA
tcctatgtgctgactcagccaccctcagtgtccgtgtcaccaggacagacggccagcatcacctgctctggagaaagaatgggggataaatatgctgcctggtatcagcagaagccaggccagtcacctgtgctggtcatctatcgagatacaaagcggccctcagggatccctgagcgattctctggctccaactctgggaacacagccacgttgaccatcagcgggacccaggccatggatgaggccgactattactgtgaggtcaagaagtccgacactggggtattcggcggagggaccaagctcaccgtccta

SEQ ID NO: 594 - protein, 106 aa, synthetic construct
  REGION 1..106: note = Homo sapiens33_640076-4B VL PRT
SYVLTQPPSVSVSPGQTASITCSGERMGDKYAAWYQQKPGQSPVLVIYRDTKRPSGIPERFSGSNSGNTATLTISGTQAMDEADYYCEVKKSDTGVFGGGTKLTVL

SEQ ID NO: 595 - DNA, 378 bp, synthetic construct; identical to SEQ ID NO: 441
  misc_feature 1..378: note = Homo sapiens33_640081-AB VH DNA
  source 1..378: mol_type = other DNA

SEQ ID NO: 596 - protein, 126 aa, synthetic construct; identical to SEQ ID NO: 442
  REGION 1..126: note = Homo sapiens33_640081-AB VH PRT

SEQ ID NO: 597 - DNA, 321 bp, synthetic construct
  misc_feature 1..321: note = Homo sapiens33_640081-AB VL DNA
  source 1..321: mol_type = other DNA
tcctatgtgctgactcagccaccctcagtgtccgtgtccccaggacagacggccagcatcacctgctctggagaaagaatgggggataaatatgctgcctggtatcagcagaagccaggccagtcacctgtgctggtcatctatcgagatacaaagcggccctcagggatccctgagcgattctctggctccaactctgggaacacagccacgttgaccatcagcgggacccaggccatggatgaggctgactattactgtcaggtgtgggcggccgacgacactggggtattcggcggagggaccaagctcaccgtccta

SEQ ID NO: 598 - protein, 107 aa, synthetic construct
  REGION 1..107: note = Homo sapiens33_640081-AB VL PRT
SYVLTQPPSVSVSPGQTASITCSGERMGDKYAAWYQQKPGQSPVLVIYRDTKRPSGIPERFSGSNSGNTATLTISGTQAMDEADYYCQVWAADDTGVFGGGTKLTVL

SEQ ID NO: 599 - DNA, 378 bp, synthetic construct; identical to SEQ ID NO: 511
  misc_feature 1..378: note = Homo sapiens33_640082-6B VH DNA
  source 1..378: mol_type = other DNA

SEQ ID NO: 600 - protein, 126 aa, synthetic construct; identical to SEQ ID NO: 512
  REGION 1..126: note = Homo sapiens33_640082-6B VH PRT

SEQ ID NO: 601 - DNA, 318 bp, synthetic construct
  misc_feature 1..318: note = Homo sapiens33_640082-6B VL DNA
  source 1..318: mol_type = other DNA
tcctatgtgctgactcagccaccctcagtgtccgtgtccccagggcagacggccagcatcacctgctctggagaaagaatgggggataaatatgctgcctggtatcagcagaagccaggccagtcacctgtgctggtcatctatcgagatacaaagcggccctcagggatccctgagcgattctctggctccaactctgggaacacagccacgttgaccatcagcgggacccaggccatggatgaggctgactattactgtggcgtgttgaagcaggacactggggtattcggcggagggaccaagctcaccgtccta

SEQ ID NO: 602 - protein, 106 aa, synthetic construct
  REGION 1..106: note = Homo sapiens33_640082-6B VL PRT
SYVLTQPPSVSVSPGQTASITCSGERMGDKYAAWYQQKPGQSPVLVIYRDTKRPSGIPERFSGSNSGNTATLTISGTQAMDEADYYCGVLKQDTGVFGGGTKLTVL

SEQ ID NO: 603 - DNA, 378 bp, synthetic construct; identical to SEQ ID NO: 521
  misc_feature 1..378: note = Homo sapiens33_640082-7B VH DNA
  source 1..378: mol_type = other DNA

SEQ ID NO: 604 - protein, 126 aa, synthetic construct; identical to SEQ ID NO: 522
  REGION 1..126: note = Homo sapiens33_640082-7B VH PRT

SEQ ID NO: 605 - DNA, 318 bp, synthetic construct; identical to SEQ ID NO: 601
  misc_feature 1..318: note = Homo sapiens33_640082-7B VL DNA
  source 1..318: mol_type = other DNA

SEQ ID NO: 606 - protein, 106 aa, synthetic construct; identical to SEQ ID NO: 602
  REGION 1..106: note = Homo sapiens33_640082-7B VL PRT

SEQ ID NO: 607 - DNA, 378 bp, synthetic construct; identical to SEQ ID NO: 401
  misc_feature 1..378: note = Homo sapiens33_640084-2B VH DNA
  source 1..378: mol_type = other DNA

SEQ ID NO: 608 - protein, 126 aa, synthetic construct; identical to SEQ ID NO: 402
  REGION 1..126: note = Homo sapiens33_640084-2B VH PRT

SEQ ID NO: 609 - DNA, 318 bp, synthetic construct
  misc_feature 1..318: note = Homo sapiens33_640084-2B VL DNA
  source 1..318: mol_type = other DNA
tcctatgtgctgactcagccaccctcagtgtccgtgtccccaggacagacggccagcatcacctgctctggagaaagaatgggggataaatatgctgcctggtatcagcagaagccaggccagtcacctgtgctggtcatctatcgagatacaaagcggccctcagggatccctgagcgattctctggctccaactctgggaacacagccacgttgaccatcagcgggacccaggccatggatgaggctgactattactgtcaggtgtggcgggacgacagccccatcttcggcggagggaccaagctcaccgtccta

SEQ ID NO: 610 - protein, 106 aa, synthetic construct
  REGION 1..106: note = Homo sapiens33_640084-2B VL PRT
SYVLTQPPSVSVSPGQTASITCSGERMGDKYAAWYQQKPGQSPVLVIYRDTKRPSGIPERFSGSNSGNTATLTISGTQAMDEADYYCQVWRDDSPIFGGGTKLTVL

SEQ ID NO: 611 - DNA, 378 bp, synthetic construct; identical to SEQ ID NO: 531
  misc_feature 1..378: note = Homo sapiens33_640086-6B VH DNA
  source 1..378: mol_type = other DNA

SEQ ID NO: 612 - protein, 126 aa, synthetic construct; identical to SEQ ID NO: 532
  REGION 1..126: note = Homo sapiens33_640086-6B VH PRT

SEQ ID NO: 613 - DNA, 318 bp, synthetic construct
  misc_feature 1..318: note = Homo sapiens33_640086-6B VL DNA
  source 1..318: mol_type = other DNA
tcctatgtgctgactcagccaccctcagtgtccgtgtccccaggacagacggccagcatcacctgctctggagaaagaatgggggataaatatgctgcctggtatcagcagaagccaggccagtcacctgtgctggtcatctatcgagatacaaagcggccctcagggatccctgagcgattctctggctccaactctgggaacacagccacgttgaccatcagcgggacccaagccatggatgaggctgactattactgtgaggtcaaggtgaaggacactggggtattcggcggagggaccaagctcaccgtccta

SEQ ID NO: 614 - protein, 106 aa, synthetic construct
  REGION 1..106: note = Homo sapiens33_640086-6B VL PRT
SYVLTQPPSVSVSPGQTASITCSGERMGDKYAAWYQQKPGQSPVLVIYRDTKRPSGIPERFSGSNSGNTATLTISGTQAMDEADYYCEVKVKDTGVFGGGTKLTVL

SEQ ID NO: 615 - DNA, 378 bp, synthetic construct; identical to SEQ ID NO: 541
  misc_feature 1..378: note = Homo sapiens33_640087-7B VH DNA
  source 1..378: mol_type = other DNA

SEQ ID NO: 616 - protein, 126 aa, synthetic construct; identical to SEQ ID NO: 522
  REGION 1..126: note = Homo sapiens33_640087-7B VH PRT

SEQ ID NO: 617 - DNA, 318 bp, synthetic construct
  misc_feature 1..318: note = Homo sapiens33_640087-7B VL DNA
  source 1..318: mol_type = other DNA
tcctatgtgctgactcagccaccctcagtgtccgtgtccccaggacagacggccagcatcacctgctctggagaaggaatgggggataaatatgctgcctggtatcagcagaagccaggccagtcacctgtgctggtcatctatcgagatacaaagcggccctcagggatccctgagcgattctctggctccaactctgggaacacagccacgttgaccatcagcgggacccaggctatggatgaggctgactattactgtggggtgatccaggacaacactggggtattcggcggagggaccaagctcaccgtccta

SEQ ID NO: 618 - protein, 106 aa, synthetic construct
  REGION 1..106: note = Homo sapiens33_640087-7B VL PRT
SYVLTQPPSVSVSPGQTASITCSGEGMGDKYAAWYQQKPGQSPVLVIYRDTKRPSGIPERFSGSNSGNTATLTISGTQAMDEADYYCGVIQDNTGVFGGGTKLTVL

SEQ ID NO: 619 - DNA, 378 bp, synthetic construct; identical to SEQ ID NO: 551
  misc_feature 1..378: note = Homo sapiens33_640201-2B VH DNA
  source 1..378: mol_type = other DNA

SEQ ID NO: 620 - protein, 126 aa, synthetic construct; identical to SEQ ID NO: 552
  REGION 1..126: note = Homo sapiens33_640201-2B VH PRT

SEQ ID NO: 621 - DNA, 318 bp, synthetic construct
  misc_feature 1..318: note = Homo sapiens33_640201-2B VL DNA
  source 1..318: mol_type = other DNA
tcctatgtgctgactcagccaccctcagtgtccgtgtccccaggacagacggccagcatcacctgctctggagaaagaatgggggataaatatgctgcctggtatcagcagaagccaggccagtcacctgtgctggtcatctatcgagatacaaagcggccctcagggatccctgagcgattctctggctccaactctgggaacacagccacgttgaccatcagcgggacccaggccatggatgaggctgactattactgtggcgtgttgaagcaggacactggggtattcggcggagggaccaagctcaccgtccta

SEQ ID NO: 622 - protein, 106 aa, synthetic construct; identical to SEQ ID NO: 602
  REGION 1..106: note = Homo sapiens33_640201-2B VL PRT

SEQ ID NO: 623 - DNA, 378 bp, synthetic construct; identical to SEQ ID NO: 581
  misc_feature 1..378: note = Homo sapiens33_640237-2B VH DNA
  source 1..378: mol_type = other DNA

SEQ ID NO: 624 - protein, 126 aa, synthetic construct; identical to SEQ ID NO: 582
  REGION 1..126: note = Homo sapiens33_640237-2B VH PRT

SEQ ID NO: 625 - DNA, 318 bp, synthetic construct; identical to SEQ ID NO: 621
  misc_feature 1..318: note = Homo sapiens33_640237-2B VL DNA
  source 1..318: mol_type = other DNA

SEQ ID NO: 626 - protein, 106 aa, synthetic construct; identical to SEQ ID NO: 602
  REGION 1..106: note = Homo sapiens33_640237-2B VL PRT

SEQ ID NO: 627 - protein, 191 aa, synthetic construct
  REGION 1..191: note = Mature Human IL-33 aa 112-270 c-terminal FLAG 10His
SITGISPITEYLASLSTYNDQSITFALEDESYEIYVEDLKKDEKKDKVLLSYYESQHPSNESGDGVDGKMLMVTLSPTKDFWLHANNKEHSVELHKCEKPLPDQAFFVLHNMHSNCVSFECKTDPGVFIGVKDNHLALIKVDSSENLCTENILFKLSETNPAFLYKVVGAADYKDDDDKAAHHHHHHHHHH

SEQ ID NO: 628 - protein, 190 aa, synthetic construct
  REGION 1..190: note = Mature Mouse IL-33 aa 109-266 c-terminal FLAG 10His
SIQGTSLLTQSPASLSTYNDQSVSFVLENGCYVINVDDSGKDQEQDQVLLRYYESPCPASQSGDGVDGKKLMVNMSPIKDTDIWLHANDKDYSVELQRGDVSPPEQAFFVLHKKSSDFVSFECKNLPGTYIGVKDNQLALVEEKDESCNNIMFKLSKINPAFLYKVVGAADYKDDDDKAAHHHHHHHHHH

SEQ ID NO: 629 - protein, 191 aa, synthetic construct
  REGION 1..191: note = Mature cynomolgus IL-33 aa 112-270 c-terminal FLAG 10His
SITGISPITESLASLSTYNDQSITFALEDESYEIYVEDLKKDKKKDKVLLSYYESQHPSSESGDGVDGKMLMVTLSPTKDFWLQANNKEHSVELHKCEKPLPDQAFFVLHNRSFNCVSFECKTDPGVFIGVKDNHLALIKVDYSENLGSENILFKLSEINPAFLYKVVGAADYKDDDDKAAHHHHHHHHHH

SEQ ID NO: 630 - protein, 577 aa, synthetic construct
  REGION 1..577: note = Human ST2 ECD-Fc/His6
MGFWILAILTILMYSTAAKFSKQSWGLENEALIVRCPRQGKPSYTVDWYYSQTNKSIPTQERNRVFASGQLLKFLPAAVADSGIYTCIVRSPTFNRTGYANVTIYKKQSDCNVPDYLMYSTVSGSEKNSKIYCPTIDLYNWTAPLEWFKNCQALQGSRYRAHKSFLVIDNVMTEDAGDYTCKFIHNENGANYSVTATRSFTVKDEQGFSLFPVIGAPAQNEIKEVEIGKNANLTCSACFGKGTQFLAAVLWQLNGTKITDFGEPRIQQEEGQNQSFSNGLACLDMVLRIADVKEEDLLLQYDCLALNLHGLRRHTVRLSRKNPIDHHSDPAFLYKVVGAAPKSCDKTHTCPPCPAPELLGGPSVFLFPPKPKDTLMISRTPEVTCVVVDVSHEDPEVKFNWYVDGVEVHNAKTKPREEQYNSTYRVVSVLTVLHQDWLNGKEYKCKVSNKALPAPIEKTISKAKGQPREPQVYTLPPSREEMTKNQVSLTCLVKGFYPSDIAVEWESNGQPENNYKTTPPVLDSDGSFFLYSKLTVDKSRWQQGNVFSCSVMHEALHNHYTQKSLSLSPGKHHHHHH

SEQ ID NO: 631 - protein, 581 aa, synthetic construct
  REGION 1..581: note = Mouse ST2 ECD-Fc/His
MIDRQRMGLWALAILTLPMYLTVTEGSKSSWGLENEALIVRCPQRGRSTYPVEWYYSDTNESIPTQKRNRIFVSRDRLKFLPARVEDSGIYACVIRSPNLNKTGYLNVTIHKKPPSCNIPDYLMYSTVRGSDKNFKITCPTIDLYNWTAPVQWFKNCKALQEPRFRAHRSYLFIDNVTHDDEGDYTCQFTHAENGTNYIVTATRSFTVEEKGFSMFPVITNPPYNHTMEVEIGKPASIACSACFGKGSHFLADVLWQINKTVVGNFGEARIQEEEGRNESSSNDMDCLTSVLRITGVTEKDLSLEYDCLALNLHGMIRHTIRLRRKQPIDHRDPAFLYKVVGAAPKSCDKTHTCPPCPAPELLGGPSVFLFPPKPKDTLMISRTPEVTCVVVDVSHEDPEVKFNWYVDGVEVHNAKTKPREEQYNSTYRVVSVLTVLHQDWLNGKEYKCKVSNKALPAPIEKTISKAKGQPREPQVYTLPPSREEMTKNQVSLTCLVKGFYPSDIAVEWESNGQPENNYKTTPPVLDSDGSFFLYSKLTVDKSRWQQGNVFSCSVMHEALHNHYTQKSLSLSPGKHHHHHH

SEQ ID NO: 632 - protein, 193 aa, synthetic construct
  REGION 1..193: note = IL33-01 - Human IL33 with N-terminal 10His, avitag, Factor-Xa protease cleavage site
MHHHHHHHHHHAAGLNDIFEAQKIEWHEAAIEGRSITGISPITEYLASLSTYNDQSITFALEDESYEIYVEDLKKDEKKDKVLLSYYESQHPSNESGDGVDGKMLMVTLSPTKDFWLHANNKEHSVELHKCEKPLPDQAFFVLHNMHSNCVSFECKTDPGVFIGVKDNHLALIKVDSSENLCTENILFKLSET

SEQ ID NO: 633 - protein, 178 aa, synthetic construct
  REGION 1..178: note = Human IL33 with N-terminal 6His tag and TEV protease cleavage site
MGHHHHHHGGGENLYFQGSSITGISPITEYLASLSTYNDQSITFALEDESYEIYVEDLKKDEKKDKVLLSYYESQHPSNESGDGVDGKMLMVTLSPTKDFWLHANNKEHSVELHKCEKPLPDQAFFVLHNMHSNCVSFECKTDPGVFIGVKDNHLALIKVDSSENLCTENILFKLSET

SEQ ID NO: 634 - protein, 193 aa, synthetic construct
  REGION 1..193: note = IL33-02
MHHHHHHHHHHAAGLNDIFEAQKIEWHEAAIEGRSITGISPITEYLASLSTYNDQSITFALEDESYEIYVEDLKKDEKKDKVLLSYYESQHPSNESGDGVDGKMLMVTLSPTKDFWLHANNKEHSVELHKSEKPLPDQAFFVLHNMHSNCVSFECKTDPGVFIGVKDNHLALIKVDSSENLCTENILFKLSET

SEQ ID NO: 635 - protein, 193 aa, synthetic construct
  REGION 1..193: note = IL33-03
MHHHHHHHHHHAAGLNDIFEAQKIEWHEAAIEGRSITGISPITEYLASLSTYNDQSITFALEDESYEIYVEDLKKDEKKDKVLLSYYESQHPSNESGDGVDGKMLMVTLSPTKDFWLHANNKEHSVELHKCEKPLPDQAFFVLHNMHSNSVSFECKTDPGVFIGVKDNHLALIKVDSSENLCTENILFKLSET

SEQ ID NO: 636 - protein, 193 aa, synthetic construct
  REGION 1..193: note = IL33-04
MHHHHHHHHHHAAGLNDIFEAQKIEWHEAAIEGRSITGISPITEYLASLSTYNDQSITFALEDESYEIYVEDLKKDEKKDKVLLSYYESQHPSNESGDGVDGKMLMVTLSPTKDFWLHANNKEHSVELHKCEKPLPDQAFFVLHNMHSNCVSFESKTDPGVFIGVKDNHLALIKVDSSENLCTENILFKLSET

SEQ ID NO: 637 - protein, 193 aa, synthetic construct
  REGION 1..193: note = IL33-05
MHHHHHHHHHHAAGLNDIFEAQKIEWHEAAIEGRSITGISPITEYLASLSTYNDQSITFALEDESYEIYVEDLKKDEKKDKVLLSYYESQHPSNESGDGVDGKMLMVTLSPTKDFWLHANNKEHSVELHKCEKPLPDQAFFVLHNMHSNCVSFECKTDPGVFIGVKDNHLALIKVDSSENLSTENILFKLSET

SEQ ID NO: 638 - protein, 193 aa, synthetic construct
  REGION 1..193: note = IL33-06
MHHHHHHHHHHAAGLNDIFEAQKIEWHEAAIEGRSITGISPITEYLASLSTYNDQSITFALEDESYEIYVEDLKKDEKKDKVLLSYYESQHPSNESGDGVDGKMLMVTLSPTKDFWLHANNKEHSVELHKSEKPLPDQAFFVLHNMHSNSVSFECKTDPGVFIGVKDNHLALIKVDSSENLCTENILFKLSET

SEQ ID NO: 639 - protein, 193 aa, synthetic construct
  REGION 1..193: note = IL33-07
MHHHHHHHHHHAAGLNDIFEAQKIEWHEAAIEGRSITGISPITEYLASLSTYNDQSITFALEDESYEIYVEDLKKDEKKDKVLLSYYESQHPSNESGDGVDGKMLMVTLSPTKDFWLHANNKEHSVELHKCEKPLPDQAFFVLHNMHSNCVSFESKTDPGVFIGVKDNHLALIKVDSSENLSTENILFKLSET

SEQ ID NO: 640 - protein, 193 aa, synthetic construct
  REGION 1..193: note = IL33-08
MHHHHHHHHHHAAGLNDIFEAQKIEWHEAAIEGRSITGISPITEYLASLSTYNDQSITFALEDESYEIYVEDLKKDEKKDKVLLSYYESQHPSNESGDGVDGKMLMVTLSPTKDFWLHANNKEHSVELHKSEKPLPDQAFFVLHNMHSNCVSFESKTDPGVFIGVKDNHLALIKVDSSENLCTENILFKLSET

SEQ ID NO: 641 - protein, 193 aa, synthetic construct
  REGION 1..193: note = IL33-09
MHHHHHHHHHHAAGLNDIFEAQKIEWHEAAIEGRSITGISPITEYLASLSTYNDQSITFALEDESYEIYVEDLKKDEKKDKVLLSYYESQHPSNESGDGVDGKMLMVTLSPTKDFWLHANNKEHSVELHKCEKPLPDQAFFVLHNMHSNSVSFECKTDPGVFIGVKDNHLALIKVDSSENLSTENILFKLSET

SEQ ID NO: 642 - protein, 193 aa, synthetic construct
  REGION 1..193: note = IL33-10
MHHHHHHHHHHAAGLNDIFEAQKIEWHEAAIEGRSITGISPITEYLASLSTYNDQSITFALEDESYEIYVEDLKKDEKKDKVLLSYYESQHPSNESGDGVDGKMLMVTLSPTKDFWLHANNKEHSVELHKCEKPLPDQAFFVLHNMHSNSVSFESKTDPGVFIGVKDNHLALIKVDSSENLCTENILFKLSET

SEQ ID NO: 643 - protein, 193 aa, synthetic construct
  REGION 1..193: note = IL33-11
MHHHHHHHHHHAAGLNDIFEAQKIEWHEAAIEGRSITGISPITEYLASLSTYNDQSITFALEDESYEIYVEDLKKDEKKDKVLLSYYESQHPSNESGDGVDGKMLMVTLSPTKDFWLHANNKEHSVELHKSEKPLPDQAFFVLHNMHSNCVSFECKTDPGVFIGVKDNHLALIKVDSSENLSTENILFKLSET

SEQ ID NO: 644 - protein, 193 aa, synthetic construct
  REGION 1..193: note = IL33-12
MHHHHHHHHHHAAGLNDIFEAQKIEWHEAAIEGRSITGISPITEYLASLSTYNDQSITFALEDESYEIYVEDLKKDEKKDKVLLSYYESQHPSNESGDGVDGKMLMVTLSPTKDFWLHANNKEHSVELHKSEKPLPDQAFFVLHNMHSNSVSFESKTDPGVFIGVKDNHLALIKVDSSENLCTENILFKLSET

SEQ ID NO: 645 - protein, 193 aa, synthetic construct
  REGION 1..193: note = IL33-13
MHHHHHHHHHHAAGLNDIFEAQKIEWHEAAIEGRSITGISPITEYLASLSTYNDQSITFALEDESYEIYVEDLKKDEKKDKVLLSYYESQHPSNESGDGVDGKMLMVTLSPTKDFWLHANNKEHSVELHKSEKPLPDQAFFVLHNMHSNSVSFECKTDPGVFIGVKDNHLALIKVDSSENLSTENILFKLSET

SEQ ID NO: 646 - protein, 193 aa, synthetic construct
  REGION 1..193: note = IL33-14
MHHHHHHHHHHAAGLNDIFEAQKIEWHEAAIEGRSITGISPITEYLASLSTYNDQSITFALEDESYEIYVEDLKKDEKKDKVLLSYYESQHPSNESGDGVDGKMLMVTLSPTKDFWLHANNKEHSVELHKSEKPLPDQAFFVLHNMHSNCVSFESKTDPGVFIGVKDNHLALIKVDSSENLSTENILFKLSET

SEQ ID NO: 647 - protein, 193 aa, synthetic construct
  REGION 1..193: note = IL33-15
MHHHHHHHHHHAAGLNDIFEAQKIEWHEAAIEGRSITGISPITEYLASLSTYNDQSITFALEDESYEIYVEDLKKDEKKDKVLLSYYESQHPSNESGDGVDGKMLMVTLSPTKDFWLHANNKEHSVELHKCEKPLPDQAFFVLHNMHSNSVSFESKTDPGVFIGVKDNHLALIKVDSSENLSTENILFKLSET

SEQ ID NO: 648 - protein, 193 aa, synthetic construct
  REGION 1..193: note = IL33-16
MHHHHHHHHHHAAGLNDIFEAQKIEWHEAAIEGRSITGISPITEYLASLSTYNDQSITFALEDESYEIYVEDLKKDEKKDKVLLSYYESQHPSNESGDGVDGKMLMVTLSPTKDFWLHANNKEHSVELHKSEKPLPDQAFFVLHNMHSNSVSFESKTDPGVFIGVKDNHLALIKVDSSENLSTENILFKLSET

SEQ ID NO: 649 - protein, 193 aa, synthetic construct
  REGION 1..193: note = Cyno HisAvi_IL-33
MHHHHHHHHHHAAGLNDIFEAQKIEWHEAAIEGRSITGISPITEYLASLSTYNDQSITFALEDESYEIYVEDLKKDKKKDKVLLSYYESQHPSSESGDGVDGKMLMVTLSPTKDFWLQANNKEHSVELHKCEKPLPDQAFFVLHNRSFNCVSFECKTDPGVFIGVKDNHLALIKVDYSENLGSENILFKLSEI

SEQ ID NO: 650 - protein, 360 aa, synthetic construct
  REGION 1..360: note = Human ST2 ECD-Flag-his10
MGFWILAILTILMYSTAAKFSKQSWGLENEALIVRCPRQGKPSYTVDWYYSQTNKSIPTQERNRVFASGQLLKFLPAAVADSGIYTCIVRSPTFNRTGYANVTIYKKQSDCNVPDYLMYSTVSGSEKNSKIYCPTIDLYNWTAPLEWFKNCQALQGSRYRAHKSFLVIDNVMTEDAGDYTCKFIHNENGANYSVTATRSFTVKDEQGFSLFPVIGAPAQNEIKEVEIGKNANLTCSACFGKGTQFLAAVLWQLNGTKITDFGEPRIQQEEGQNQSFSNGLACLDMVLRIADVKEEDLLLQYDCLALNLHGLRRHTVRLSRKNPIDHHSDPAFLYKVVGAADYKDDDDKAAHHHHHHHHHH